European Patent Application EP 4 534 671 A1, published April 9, 2025. Title: Antisense Oligomers Against Monoamine oxidase B and Use Thereof. Applicant: Institute for Basic Science. The sequence listing filed with the application follows.

SEQUENCE LISTING (41 sequences)

SEQ ID NO: 1 - RNA, 20 nt, synthetic construct
  misc_feature 1..20: note = Synthetic Sequence
  source 1..20: mol_type = other RNA
ggaagattccagaggatgaa

SEQ ID NO: 2 - RNA, 20 nt, synthetic construct
  misc_feature 1..20: note = Synthetic Sequence
  source 1..20: mol_type = other RNA
ctcgtgtgcctttgggttca

SEQ ID NO: 3 - RNA, 20 nt, synthetic construct
  misc_feature 1..20: note = Synthetic Sequence
  source 1..20: mol_type = other RNA
agctggagaggcctgtgatc

SEQ ID NO: 4 - RNA, 20 nt, synthetic construct
  misc_feature 1..20: note = Synthetic Sequence
  source 1..20: mol_type = other RNA
ggtcaagtgagtgagcggat

SEQ ID NO: 5 - RNA, 20 nt, synthetic construct
  misc_feature 1..20: note = Synthetic Sequence
  source 1..20: mol_type = other RNA
tatgtgaagcagtgtggagg

SEQ ID NO: 6 - RNA, 20 nt, synthetic construct
  misc_feature 1..20: note = Synthetic Sequence
  source 1..20: mol_type = other RNA
ccaacccagaatcgtatctt

SEQ ID NO: 7 - RNA, 20 nt, synthetic construct
  misc_feature 1..20: note = Synthetic Sequence
  source 1..20: mol_type = other RNA
taaatatgtggaccttggag

SEQ ID NO: 8 - RNA, 20 nt, synthetic construct
  misc_feature 1..20: note = Synthetic Sequence
  source 1..20: mol_type = other RNA
agggttctacgccagccagt

SEQ ID NO: 9 - RNA, 20 nt, synthetic construct
  misc_feature 1..20: note = Synthetic Sequence
  source 1..20: mol_type = other RNA
ggctaaatatgtgattagtg

SEQ ID NO: 10 - RNA, 20 nt, synthetic construct
  misc_feature 1..20: note = Synthetic Sequence
  source 1..20: mol_type = other RNA
ttcttttcttactgaagctc

SEQ ID NO: 11 - RNA, 20 nt, synthetic construct
  misc_feature 1..20: note = Synthetic Sequence
  source 1..20: mol_type = other RNA
gtctaacaatagctctttcc

SEQ ID NO: 12 - RNA, 20 nt, synthetic construct
  misc_feature 1..20: note = Synthetic Sequence
  source 1..20: mol_type = other RNA
atcttgtctatgtatccagg

SEQ ID NO: 13 - RNA, 20 nt, synthetic construct
  misc_feature 1..20: note = Synthetic Sequence
  source 1..20: mol_type = other RNA
ttggcaaatgttaagggcag

SEQ ID NO: 14 - RNA, 20 nt, synthetic construct
  misc_feature 1..20: note = Synthetic Sequence
  source 1..20: mol_type = other RNA
gcagtctcctgggttacata

SEQ ID NO: 15 - RNA, 20 nt, synthetic construct
  misc_feature 1..20: note = Synthetic Sequence
  source 1..20: mol_type = other RNA
atttgtctagtgatcattct

SEQ ID NO: 16 - RNA, 20 nt, synthetic construct
  misc_feature 1..20: note = Synthetic Sequence
  source 1..20: mol_type = other RNA
ctttcaaacaacaaagggta

SEQ ID NO: 17 - RNA, 20 nt, synthetic construct
  misc_feature 1..20: note = Synthetic Sequence
  source 1..20: mol_type = other RNA
ggtttcaacctatctccaat

SEQ ID NO: 18 - RNA, 20 nt, synthetic construct
  misc_feature 1..20: note = Synthetic Sequence
  source 1..20: mol_type = other RNA
gccttgtcttcacaaacatt

SEQ ID NO: 19 - RNA, 20 nt, synthetic construct
  misc_feature 1..20: note = Synthetic Sequence
  source 1..20: mol_type = other RNA
caaacagcccttgttaagca

SEQ ID NO: 20 - RNA, 20 nt, synthetic construct
  misc_feature 1..20: note = Synthetic Sequence
  source 1..20: mol_type = other RNA
gcaaattttaatcactccct

SEQ ID NO: 21 - DNA, 20 bp, synthetic construct
  misc_feature 1..20: note = Synthetic Sequence
  source 1..20: mol_type = other DNA
ttcatcctctggaatcttcc

SEQ ID NO: 22 - DNA, 20 bp, synthetic construct
  misc_feature 1..20: note = Synthetic Sequence
  source 1..20: mol_type = other DNA
tgaacccaaaggcacacgag

SEQ ID NO: 23 - DNA, 20 bp, synthetic construct
  misc_feature 1..20: note = Synthetic Sequence
  source 1..20: mol_type = other DNA
gatcacaggcctctccagct

SEQ ID NO: 24 - DNA, 20 bp, synthetic construct
  misc_feature 1..20: note = Synthetic Sequence
  source 1..20: mol_type = other DNA
atccgctcactcacttgacc

SEQ ID NO: 25 - DNA, 20 bp, synthetic construct
  misc_feature 1..20: note = Synthetic Sequence
  source 1..20: mol_type = other DNA
cctccacactgcttcacata

SEQ ID NO: 26 - DNA, 20 bp, synthetic construct
  misc_feature 1..20: note = Synthetic Sequence
  source 1..20: mol_type = other DNA
aagatacgattctgggttgg

SEQ ID NO: 27 - DNA, 20 bp, synthetic construct
  misc_feature 1..20: note = Synthetic Sequence
  source 1..20: mol_type = other DNA
ctccaaggtccacatattta

SEQ ID NO: 28 - DNA, 20 bp, synthetic construct
  misc_feature 1..20: note = Synthetic Sequence
  source 1..20: mol_type = other DNA
actggctggcgtagaaccct

SEQ ID NO: 29 - DNA, 20 bp, synthetic construct
  misc_feature 1..20: note = Synthetic Sequence
  source 1..20: mol_type = other DNA
cactaatcacatatttagcc

SEQ ID NO: 30 - DNA, 20 bp, synthetic construct
  misc_feature 1..20: note = Synthetic Sequence
  source 1..20: mol_type = other DNA
gagcttcagtaagaaaagaa

SEQ ID NO: 31 - DNA, 20 bp, synthetic construct
  misc_feature 1..20: note = Synthetic Sequence
  source 1..20: mol_type = other DNA
ggaaagagctattgttagac

SEQ ID NO: 32 - DNA, 20 bp, synthetic construct
  misc_feature 1..20: note = Synthetic Sequence
  source 1..20: mol_type = other DNA
cctggatacatagacaagat

SEQ ID NO: 33 - DNA, 20 bp, synthetic construct
  misc_feature 1..20: note = Synthetic Sequence
  source 1..20: mol_type = other DNA
ctgcccttaacatttgccaa

SEQ ID NO: 34 - DNA, 20 bp, synthetic construct
  misc_feature 1..20: note = Synthetic Sequence
  source 1..20: mol_type = other DNA
tatgtaacccaggagactgc

SEQ ID NO: 35 - DNA, 20 bp, synthetic construct
  misc_feature 1..20: note = Synthetic Sequence
  source 1..20: mol_type = other DNA
agaatgatcactagacaaat

SEQ ID NO: 36 - DNA, 20 bp, synthetic construct
  misc_feature 1..20: note = Synthetic Sequence
  source 1..20: mol_type = other DNA
taccctttgttgtttgaaag

SEQ ID NO: 37 - DNA, 20 bp, synthetic construct
  misc_feature 1..20: note = Synthetic Sequence
  source 1..20: mol_type = other DNA
attggagataggttgaaacc

SEQ ID NO: 38 - DNA, 20 bp, synthetic construct
  misc_feature 1..20: note = Synthetic Sequence
  source 1..20: mol_type = other DNA
aatgtttgtgaagacaaggc

SEQ ID NO: 39 - DNA, 20 bp, synthetic construct
  misc_feature 1..20: note = Synthetic Sequence
  source 1..20: mol_type = other DNA
tgcttaacaagggctgtttg

SEQ ID NO: 40 - DNA, 20 bp, synthetic construct
  misc_feature 1..20: note = Synthetic Sequence
  source 1..20: mol_type = other DNA
agggagtgattaaaatttgc

SEQ ID NO: 41 - DNA, 115841 bp, synthetic construct
  source 1..115841: mol_type = other DNA
aatatagcggctcgccgaggcgctggtgcacgggggcagcgcgcagcaggccggcgggcaggcgggcgggctggctggcaggcaggactgggatcgaggcccagaaaacggagcagcgggcaccagggaggcctggaacggggcgagcgccatgagcaacaaatgcgacgtggtcgtggtggggggcggcatctcaggttagtcgcggctgtgcgccctccttcctcttcacgcgctcggacaggtggctgcctgggggagacgcggggggcggccgtggggcaggggctgaccctggagtccccagactgtccacgcacgggcagggctctagtgggtccagagcgccgtgcactgaaccctcctttgggggcaattttgggtgcgttcccggacgcagaggccagaggctggaagcctgttgcagctctggggccagactttgaacttctcccccagaaggctgctaggccttcgcttgctggaattttcgaagccagggaaaaggggtggggaggtggcacaaaggtcagtcatttgctccaacttgacctggacactccgcaccctcgcttagagcaagcatgcaccacatcgtattgttgtcctggcgtcaggaaaacgaccttgaacagaagaggttggagcctggccaatcgattgccaaagactttccaggccctcctgattctttgaggttctgtgattgtcacggatctaacttgaggctgcagtgtctttttggcaaatgcctgttttcctcttatgcctctcgcacccccactccaccccaccccactcctagcgcagggtggccaagctgcagctttgctctctggcctagcccatatttggcaaggatggggacagacactaccccctcagccacacggggctgtgtacataccaagggcaccgaaaaatagaagccagaagaagggatgggggtagtggtggaacttaccctctgtggaggatcaggcagatcctatgggatagggtcaatgggaatcaatgatgctctcagcacagcctgtttaatggccccctgggcatgctttggcccacctcctaacgctgcctagtacttgagcagtaattaggacacctccagacccgtggatgcattgtctaagacttgccttaaggagttctcaagtggcctttgggaagtagaggttggccttgctccctgccaggagggcaggacagagttgttctgactctcctgtggctggagaaaaaaccaaggcattggatgtttggtgctgaccatggtccagtcctcctgcctctgctccagcctttctcccctttgggtgggatctcaggctaccacatctgtctagcaggctctggtgagctcgcccatgccaggccctgtgcctggtgttgcaggtacatagatgcgtaatcacaacatgctgaggttggccaaggctgtgtataaattcagttttctttcagtatttttgacatcttctctcctagaggaagttggacttaaaagcatacctacttaggtgttttagaaaatattactaagtgcctcttgatgctgccttgcatagcaccccatcttacagaagctgaagtttctcttttcaggcccccgaagtcattttctcactaaagtatgcccaatggattcagatttttctattttcccttcatgatttgtccctttctgattcatactccacaccttcaggttcaatcacattactcatgttagactcatctggaaaaggtagataagggtttaactatttttgcaagcagtggtgaaacctctgcattcatcctcccgaactctgatcaaaacaaggtactgatgagtagatctgacttttctcaagaacattccacggaataggcattgttctaagaaccaagaaagcagccttccaaggcccagtcttactcaattgcttcatctgctacatggggataacaccagttagtcactgctggattacagggcaagtgaaacaatgtgagtaaaatagctttgcagagtctgaaatatggcacaagcccctcaagagttttacccatttattcagacaataggaattgagggaggctgtgtaggggattcaaaaatggatcatgttgttcttgccccggaagacttgtcaattcaagaagggtgatgggatactcagacaatacaaggtagaaggtggtgcgtgccatgggaggggtccattcattgattcattattcattcattcaatgaacatttacttcctgttccacattttgtcccaaaagaaataaaagatgatttatacagggccattgttcctggggccctcacaagctgatgtggaagacagtcaagaataattactactctttggcatatgataggtgctttaatagtgcatataaaaaattctagggaaggtgattggagagaacatcaaactctgtctgagaaaatctaagaactcacagagttggtgacatctgaactatgtcttcaggaatgaatatgaattcaccaggggactagatgaagaaagcatttttaaactaaagagcagcttgtataaaaccacaaatatgtgaaagaacatgctaacgtgtaggataacttaagaacttcattgcggagagttgccagaggggtctggtgggagagaaagctagaaaagtcagttgggatgaattatggggaggcttgtatatcagaaaggtttagctctttctgtgatcaatgaatagcactgatgattttttattcagagtgccatgcatcaaatggcgtgtgtcacatctgatggtgatattagcaaaaagagggatatgaagaagagggagagaaggttttgggaaaagataggacgtctagagttggaggttctgggaggacacccagggagagaaatctagcagttggaatgaaattggggttacaaatgtgtacgatagaggttttagtagatgaaatggccaaaatcaagagtgtagtgtgtagaattttcgaattagtaggtgaccaacacaatgatttatgtttaaaagtctctggatttgactctgcgttctaagctttgttaattattaaacttgggacattctggcaattccctgataatttttaaagctgtcagcaaattttaatcactccctttgggataaacagagacatactgggaggatagctggttaatacataactttcttttttgatgttttaaaagttccaagatagttgtagactaactttttagaaatgtgtatggtgtataaatgagtatgcactgaaatctcttttacccaaggggcagatcatctccagagacttggcagagcaatgacatctcccacatggaactggacagcagcacgttgcatctgtcccgcgtctctcagttttagtgtttgggtgggtggaaccatggaaactatcttttgcaattctggaatagttcttgttcaatccccaaaataaaaactaaaaaaggcaacttgaagcagaaacaagaaagttttggccagacttaggagaggagatttggtcatttgagggtggcaggcacttgtttgagatccctggaagtgttggaaccagacttccaaattgtaaccaacacctggcaggtgatctttgtggcagggagagcaagcctggctgcaggctagtggtactggctttggcagggaatgtcagagatggctcacaaggggttatgagttgaggtgtgtggtgggcagatgtggcccatatgttaatggcaaagcctctttctcacctttggtgaagaaaaatggagaacttccctgggctcctgtaacccacttgaatgtcctaaaaaataataattatatagatatgcctgaaaatttgtatatcctagtcaaggaaagaatacacagaggtaatacagcaatattaaaagaacatacgatttatcttggaaggttgagacgggaggattgcttgagcccaggagtttgagaccagccctggcaacgtaatgagacatggtctccacacacacacacacacacacacacacacacacacacaaaggctgggtatagaggagtgcacctgtagtcccagctactctggaggctgaagtgggaggatcacttgagtccaggagctcgaggctgcagtgagctatgatcatgccattatactccagcgtgggccacagacaaagactgcctataaaaaaagactgggagggggagaataggcttagtgtcaaacacactagttatgaatctcatttcttatgcttacctatgtggaaccttaaaaggtacataacctccctgtatttcagctgcctcatctttaaaatgagactcataatgccttcctggccggcttgtttcaaggattggaaagaatgcacatgtaggaccataaacagtgatcacttcggctttggcttataggtgccttactctacctttttggaaatatatccttgtttgtcctgtagagtttttcaatctaagggagcaaaaacaggcatttctatgtaatcacttcttttcaccaaccaataatttttctggatgtgcagcatagataaggtggcaacaggacgccatgtatacatgtgggcatcaggagagactcgcctgacttcagcctcatcctggctcagccaattcctttatccccccgcaaggggcctgaggaactcaggctcactttgggctctgagacccactgggttccgcttcaggagaaattctggaagtcttagatctgtacttcagcctcacctcaacctggctattattccaattctgatctggtcttcatttcagccatttgattcctgtcttaactacaatagaagataaatgcattaataacaaatgatattatttatttaataatattatttaataataaatgataaaaaggtagcatatcaagcgttatctacatgctgtacaaggtgttaggagcttgattagaatgacaaaagctctgtgaaggttaagaatgacaaagccttgttctttctgcttgattctaacacccctgggacacagtgttggggccggttggtgggctgtgtgagtagagccagttgccactagagtcacaatttctaggcccccatgtgtcctcagaagtcaccagggcaggtttaaggcttggcttggcattgacaatggtcacaattttcttctcctctgactgggtattgaggtctaggctccctgccatacattcaggggcagtggtggagcataggggttaagagcatggtgtctaccctggttccaccactaactagctgtgccaccttgggcaaaatagttagttaaccttcccatgccttacttttctcatttggaaatggggataataatggtatctatttcacaaagtggctgagagaattaaaggagaaaatacatgtagagtgcttggaatgtggcttggcatttggcaggcacacaatagatattgatgattattgttcatcaggctgacaaaatgtccactagcaactagtggtctgaagtgccagtgtgccagcttcctcactgtcaaactttgggctgaggaagtggtttgtggctgtgcatttgaatgcactgacacacacacacacgcgtgcatgcacactcggagaacattagcctgtaacagagattctgcttccaagccctgttttcttggcttgtatatgatttactaacacagatgatgtgagaaagtcagcagcttaatttaaacaaaaggctttaactctaattattttaatatgtattttaagagataaatatgtcagaaactataaatgcaaaacatttgtatacgaagaggaaggaagataacacagctgttaaacacaaagggcattggaggcctgggacttgggctcaaatcccatctgttcccctaaatgtggagcttgggcaataggggtggcaatagtaacaggttagtttttttgtggagttcaattacagatgattttcatttttttccattttctgtaatttacagattttcacaacaaatatgtattatttctgcaactcacgtttccagaaacaccatactcttccctctccaaaaaaattcctcaaagtataaatcaccatgatggaatgtgactgcatctttcatttatatcagtggcttttcttcttaaaaatatttgagggaatttttgttattaataagtgtggttattggccaggcatggtggctcacacctgtaatcccagcactttgggaggccaaggtgggtggattgcttgaggtcaggagttcaagaccagcctgaacaacatggtgaaactccgtctctactaaaaatacaaaaattagccaggcgtggtggcgcatgcctccagtccgaagctacttgggtggctgaggcaggagaatcacctgaacctgggaggcagaggttacagtgagccgagattgtgccactgccctccagcctgggagacagagtgagactctgtctcaataaataaataaataattaataaataaatgtggttattaattcttcaatttatccttctgcaaaagatgccctgctagatatcaaaagctctttcaaagagcttgtctcttcaatttgtcttggtacttcttcagccaagtttcttcaatttttcttggtacttgaaaagcgggtgagtgttcctgggctaactcctagaattctcaataaatgttaactttgttatttgtacaagtcactgggcagtactcaattgagggcaccctggaatcatgcaagatcgaatacccttgaagggtgcaaaagtgagccaaattgaggggccacgttcaggtgtaatatgtgtctgaagaacgagtgttttcagccccacaagagaatgctttggaaatttgctcaggttaaatgtgtaccattgtgcttttgcaagaatctcattcgctgggcttaacttattagtagtgtgtctgcataaaagttgttatttcccctaagaggaggccataatggtataaaattccttcctgattttgaatattcaaggaacaaacttagaagaccaagctaaaaaatactttggtttaatagaatcattggtgactgaagacggaagcatctttagagttttacctactagttaagatcgcctggttttgcatccaagaaaaagcacatttagagagtgcaaagggctggctccagacctcacagccccttcttttgaataaaattattgtcctggaggatgagccctcagccttaggagaaaatgcaaacagaaggacaacctgatcaaatggtgctgggtgagaggttagaatcactaatactttgaatgcactatttctactttctgttttcatgctcacaaaatggatccatctttggcctcctctgttaactcagtaaataaagatacagaaagccaagtccctgttagcaatgtttcctaagtcagcatgcatttatttactgaaggaaggtatagaaaaagagtaagactaagttcccagcctcaggaaacttaaaatgcagatggagacacaagactagcacatacatgcaataaggaacaattaaactaatgtataattgaattctgaactgtgggacccaaggactaagttagaagaatcattaaagaccccaggagttggagaaggtctcattaagggagtagaatttaacagattctgaagaacagtccaggtttgggagggtagagaagagagaggctttaaagatgagaagaatcatttaaatcatagggccagagacttcagttagcaggtgatctttatatttacaggacagtagaaagtccagcttgtctagaataaaaggaaggggagacatgggaaggaaagttagtaggaggggggcaggatccaaaaacgagcaattgaaaaacaaagtgaaaagttaggttttcctgtggtaagaaatagggagccattgacagtttatactataaagataaggtggatggtcgtgtgcctgataaccagggaagccaaaacatggatagaaattcaggaaaggattgagaggtgatcagctgattataatgtattgggttattctgaatgcccaagggaggtttcaagagaaatggggatagaaagaagggaagaatgagtagaaggaggtgtccaaagttgcacttggctttcttcactgtcttgctggcagcctatccagaaaagaagtatcacaaacaataattagttgtaatttaatgaagttgtaggcactccataaaacatttaccactgttactattgccacctatattttatttttgcaaacttccctccaaagttttatcattgggattgaaggacttgactgtatttacattttttcttctttaaaaaactaaaaacagagattttcttcccaagggctgtgacccagtttactaaatgataaaacgtgtatctctggcaatctcaaacacaaaatgaatagttcatcttatttgttatataaaaactgtcggccgggtgcagtggctcacacctgtaatcccagcactttgggaagccgaggcgggcggatcgcgaggtcaggagaccgagcccatcctggccaacatgaagaaaccctgtctctactaaaaatacaaaaattagccgggcgtggtggtgggcgcctgtagtcccagctactcgggaggctgaggcaggagaatcgcttgaaccagggaggcggaggttgcagtgagccgagatggcactactgcactccagcctggcgacagagacagactccatctcaaaaacaaacaagcaaacaaaaacgaacaaaaatgtcatttaaaccttttgttttgtgagagaggggcaccatcagaaaacatcttcaggtaggtctgacctttcaaatgttagtcatcttaccatagtctccatttaatggcatcttaaatgtcatatactatctaatttccacttcatatctgaaatttgagctcttgatcttatgttatgcatctcttagctaggccatttttaattctactctcctcctcaataacatttatcagaattacacaatgatgaaaatgtcctactagatacttagttttatttgctctccttctagcctaaataatcgtcccttttgcttaacctctccaacatttttaatgattcttttaattgaatttggaatccttacttcatattttgaagttgggctactttttattgctgtgatcccagtggtgtgtgtgtattaaattgtgtattgataattatgtctttagttatatctcatttctttgggttattttccagttttctacattaaagaaacaagctcattggaagagcttttgttatccagcaaagcatcttttttcagaaggataaagttaagaattaataaccaatttagttaataaccaaaattacttcaaacatttggtaagaagaaaggccactgatagaaatgaaagatgcaatcacattccatcttgatgatctacagtttgaggacattttttagagaggtgtgagtatcttttttaatagcatgaatgcagaaataataaacatttgttgtgaaaatctgtaaattatagaaaatggcaaaaagaaaatgaaaatcatccataattgaactccataaaatatttaccactgttactattgccacctatattttctttatgcaaactttatgttgtatttactgtacttatttgtatcccctttaaaaataaataccaacatgttatgaatgtttacctatgtcttaaatgttttttcatgattttataacattagttcatatgattgtatcacaacttgttgaatcaatctcctattgctgaacatttgtgtttttttcaaactttctgctattttcaacaaagctgttatgaacctaaattgttgtacataattctgattgtttctttaggaaatttccagagataaatgttagaaattcttttaaggcatttaataattatagcaaaattgtcgcccaagaaagttttaccaatttaccttatgatggaattgtaataatggacttcttagccatttcaataggaaaccaacatttcctccccacccaacgatcccccagacagtacagagataatcaagattcttcaccagtttgtagtcgtaatttaatgaagttgtaggcactagaaattaaaaatatcttcagttttgtaacattttagtggtggcaagtaagttttgctctctgtaacatgcaggaaagctgttttttgcaattactacgttatgcctaccattatctactgggaacatatacttttatagtacttttaaatttattgggtaccatctagcctgtgcttccagaagtttgccatcattaattagataactgttgtgtttctatgcagaaaagaaaagaaaatagtcctgtaacaaaccattttctatgattaattatttttacccatctagataaaacatgagtatagcctttgttcacagcctattgtaacagctgatcaaacagctgtttcatgttttacattttaatttcctctgtattttgcattcaaatcctgtgatagagtttaatttatttaggaaacccataagatatagtcgactgtttcagaatagcccttttatgctgtgccagttagtggaaatcaaacagcccttgttaagcaccgatgataaatacacataagggtgtgcactaaaagagttgtcctcgtttcatcaaatgtatttccctatgtcattgtttctgcagggagaaaaagaaatttgttcattcgttgattcagtcattcaataaacccttatcgagtgccctatttaccaaacattgggctaggtgtgggaatacacagatgggtaatacatgtgcccatctttcaggggtacaccaagcagaaggaggcagacatgtacaggtgaatgttctgaggggtggtgggtgctgagaaagacatgcttatctggatcagatgagacagagaagaggaggacagcagcttcacctcaagggcctcagaggccctgaaggaggatttggcaatggaatttactggagaggtaaccagcaaattcaaatgttcttccttgaaatatagctttaagtagttggaacttaaatctatattctaatgtacatagagtgttgaaatttcactttcactctttgtatagtggatgttatagtaggctgtcccactaccttcaggacctgctgagagtgttggctgctgctggctcacagccaagtccctctctgaaagtcacccttgactgaagggagctgactaacccaggccttcgtaccctcttgcttcaatccaggataactctgaaaggccacattagcctgagagttcactgtaggactgattgatttctctgttgtgcttgcatctctcagttcaactccttcctttgcccaatcctgcttcctttcttcatacatgttgaaccccgataaagcttctatatgcaaacccatctcagaggctgcttaccaggggaccctaagctagacagaggatgactgaacagcatttttgctcagcgtgtcacaagatgttctaatcatgaagtttcagacagttggaggaagaagcaattaaagggcatgacctttcccatgttcttttcttttctttttctttctctttttttttttttttttttttttttgaggtggagtctcactcagttgcccaggttggagtgcagcggtgagatcttggctcactgcaagctccgcctcccgggttcatgccattctcctgcctcagcctcccaagtagctgggactacaggtgcccaccaccatgcctggctaattttttgtatttttagtagagacgcagtttcaccatgttagccgggatggtctcgatctcctgacctcatgatccgcccgcctcagcctcccaaagagccgggattacaggcgtgagccaccgcccatgttctttaatggcctccaccaaggatgcaagaggccggtagggcctggagacggtgcttagtctcatcagttctggataagcactctttggtgccctgagagcccccaagtaagggtgaaaggtagaggttgatcactatgctggcccaaacactctctggggaatcccaatctcttaccactctgtgtgctgattcagagctgaaatttagagcctccgatctggaagtgctcaaaatatggattccttcttttactggaggaatccgtggcagtacagccaagagagaaattatgaaacagccctaatctgtgaagactggatacagaagtttggacgctgtccatctattccaagccaccattttggatccagctcagattctgggttcttggaaaaatagtgctgttggcacacacctctattctttcccttatcctgtgaccattttatgcagcttcctgtaggatttctcacagggtgttgaaaatgctgaaagtgattataaaaaaaatggacaatggagttcttgatggataagggagaaagggaagttgtgagggagcaagctggttcatagattcaaatggagatgttaatagattggaggtctttgtgtcattaaagaacatttatattagagcaatttgagcaggtgaactagaaagataggaaatcatgattgtgagggggtgttctgtagggttttgacgatgaaccttttgatatgtgctacttggaaataaccattttttaaatgagttgcaacattttgaatcagcatgtccagagatttaattttctatgtgattcaaaaaatgatgtaagagtcagaaaaatgattttctttcattttattttctatttactaatctgctattggttttacaacagggcagaagagacaactatccatttaatctaagtttagagattggcagaaaagtccctctgttttattgagaaaggcaggaatcatacactttggggtcctaaagattctaagcaggtctctgttaaaattgcatgcaggtcactggggagctaacccctcaactgctgatttgctatgtgagtgatgtacagcaggctggggaggggaaccaaagcaaggtgctcaaactacagcaatgcaaagcagttgggagacataggcagcctttatctcccagctgtttttcttgaagatgattagaaaagcatagaaaaaagtcagagggtgtacaaaatttagcgttatttaaagtccagtgggaacagcactttgttctattccaaaacaaattataatagagagagagagatcttgtccttcccacaccccatcaaactacactttatgcagctagaccattagtgttatgataccattagcactttgagaattctgttctctgactgaaaaagaaaaagcacattgtttatggaagggtctgtaaaaggaaattgcgggctagttttcaaccctgtgattcagcctcatatatttactatctacccgaaatctttgccggcaacatgccattctatccccgtctgtctgctacgaggctatcatttagaaaacattaactgaatgcctcctgtgtgctaagtgctaggaatgaataatcaggttccagttcaacacattcacacacacacacacacacacacacacaagaattgatgtgaaattacgttttctgtgcttatttatttttggtgcatgcacaaaaatgtactttttaaatgaaagaagcctctcggtgccgtgaaagagctttacctttggacaaagttagaatggatgctaagatcactttggctttgctttccaagtctctgtcctctgctagcttttttagttttattcatgggtggtatgatattcctggccttataaggggtataagtaaaatatcatacttgccttttatgttatcagaaattgggctgcacacaggaaccgtcagtgtctgaaaggaaatcacatggtcctagttgataaaaggcagaacatccaaaatataccacccgtgtcctgcttctctccccttgttcctttctctctgatttcatagagaatgtgtccaagggggaaatgagttttctgtagataaatcagttggccagtccacagtattgagcttccagtggacaggtctgagaaatggggaaaaatacaaagaggttgagatgacagtaagtaggaaaggtaaaagcattttgcatgtagaagaaaaatcatttggggtgtgcacttgctttatttctgggttttagtttgtgatcagaaaactagcagaagctgatgaaaataggaaagcatttcttttctcctattgtgttctttaaaaaatatatttcgccaaacagatattttataaaatctggcttccttccccatagataaattcctttgaaaggagtctgtaggtttaaaggttgcttcagaatacatttaaaattaatctttaaaattaaaggcattagtgaattttaaaattccattgaatatatgtttatgtgtaaagatgtttgaatactttttcttagggaaaaaagggattttaaaaaagaaatattagcacttagaatttaaaccagcttttaaatgatacatcctatatataaattttagcatcatttttcaatatttttaaaatgcaatgaagatctcaatggcaggtgaaaaatgatatctgcaagtgattttttaaatgggagcttattcaattttgtaattatagctgtatgtgaagaacaaacaaaatacatgtgcaaaatataataacagcaatatctgcctggtatttctaaaggactttggttacatataattcttgtacgcatgataagaaaaggaatgttaatttttaactcaacaaatacagcgttcctataaggtggtctgtacagtatattggtttgtataattcacacattaagtgaaaggaaagaaagagatgaggagtggaaacacttatctcatactcttgtctagttgaatattgttttttccatctttgacatttgaattttgtagtacagtgcagtatgaggtgtttaaagcctataaactgttatttaactaatactgttttctaaaatactttccatgatctaagaaaataatttctagtttcttgggctatgtattaactgggcattctaaaacgtcacttctcatcactcccatgatagtacaatttcctgcttccctcctaaatcgctagtgctccaccagtctcctttgccagctcccttcctttgcctgctccttcttctttggccaccaatgtttccggtttcaggaagtggaaccatattctggccaggtttccagccaagagtcttgacatttgtagcagacattgcagggatcctaccaaatctccttggcacttattttcatacacatgaacttaaggcctctgtctgatgcaagtttttgcctgcaggctttctctggccactggagctcctcttggctcaaacccaggcaggtgagcagtgcgggtggggctaatgccccccgaaaagcagccatgagtctgtgactaacatgatttgatggataagtaacccatcttcctcatctcttaggatagctaaagtgtgttccacactgtctcccagatttccccacagttgcccacagtggtaaccacttaactgtctccatgccccttctggatctggtgttcctcacgtggaccactgtagttcccagagtctgctcatttgtgtcccatcattcggtctagcccttctccagtccattctgtttttctattatggtaaaatatacctaatgtacaatttactgtattaactgttttaggtgtacagtttagtggcattaagtacattcacattgttgcacaactatcaccaccatccatctccagaaccgttgcatcttctcaaacagaaactctgtacgcattaagcaataactccccattcccttcttccccagcccctggcaaccatcattctactttctgtctctatgcatttgactgctctcagttcttatatgagtggaatcatacagaatgtgtccttttgtgtccggcttatttcacttagcataatatcctcaaggttcatccttctagttcattcttacaataaaggaagtacaacttgtgaattgggaaaaagcagattggatattttttagtcacaaaacatatttattgtcagaagtgaagcaaacaaagttgttcaaagacaaagctaaatatttgtcgaacttcacctcattcctgccctcctgaggtgacctgtgttaacagcctggtgtatttcctttcacacgtttctcctggaagggcaatttttctaaaatgtaaatctcatgagatttactcttctgcttcagatctttccatggccctccattacccccaggataaagtctgaaatgatggttatggcccagaaacactgcagacctgaacttggcctacttcggatgccttgtttcccgtggctcttcctagggcctgtagctacactgatccactttgaagttctcgaataatctgcaacctctggcctttgtacctgcttctgtcacgtgtagtcttcctagttctcctccctcccacccctgacctaggtaacttttgatcattcttccaaatatattttaaaattcacttttaggggtccttcctcttgtctgacagacctgtgtgaactaccttagcgcctgcagccagaaaaaaaaaaaaaaaagcttttgggcaaagagtcagtcactgtagttcaaataaacaatggttgttcgtagaagtgaatgaggagggaatatgggtataacatcgacaatacctgctacaacatttttcatgaaaacctctgaatcacttgaaaaagtaatgacaataatcaatcttattgagttctaaaattttatcttcataagatttttaaataatagctttgttgagatattattcacatacaattcacccatttcaaatgtacaattcagtggattttcatagattcacagggtcttatgatcatcaccccaatgtaatttttgaacatttttgtttccctaaaagaaaactccacatcccttagcagtcattcctcattccccatcaccaccgtcagtccctcagctccttacaaccattaatctactttctgtctctagatgtttgccaattatgaacattttatacaaatagaatcaaacactgtgtgaccttctgtgtctggcttctttcatttagcatcatgtcttcaagattcatccatgtggtagcatgtatcaatatttcattcctttttaaggccaaataatattctataatatgggtgtgccataatttgtttatcttttaattagttgatggacatttgggttgtttccactttttggttattatgaatagtgctgctatgaacattcttgtacaagtttttgtgtggagatatttttatttctcttcggtatatacccgggagcgaaactgctagatcataaggtaactctttgtttaaccttttgaggatcaccctcttaagattttaaagtacgatctgcagtgatttactgaatgtcacatagtgcaggtacacctacaaagccatcattttgtgctgcctcctggatagagggtagagatgcctggattactgggttgcctgtgtctctcatatgcttttctgagatggttggtgctgggagagatcctttgggaaaaactcttagcctgttcagcttctttaggtaagatgctgtcctgaggctgacccagttctgtctagttctgacccagttccaaacattaagtagagcatccatgtaccatgccaagccatacccttcccgtcctttaaaagctgactctgggccatcttgagtgttgaaatcaaacctaaacctcctctatgtagttaatcccaaagcccaaataagatatcatattggcaggaataaatccactcatcaaagtttatccatccattgtttgaggtgattgtttcctggattgtaggtattcctggaaaataatgtgaaacaaggtaagcttccaggaatgaaatgcaaactaaatggaaattaagacacattcataaatgtgtctcacaagaccaatgaagctaaaacatttatcactaagaaaatgattatccaaaacaattatcctaaacagtaagcatttggtaagtaatatcatatatacgtatacagataatgtatgtatgtattgtatatatatttatatgtttataaaataaacaaaatgcttcacatgaaaactccaactagagaaaatacgtatatatttaatgtgtgcatatatgaaatgcgtttacttacatgaatatatttatatatacatatattttgacattatgtttaacatgtagtaagtattctccttagcctagagttacagatagtgatgccaagttcagtcccttaattgatgaacaataattatgttgtattcatcagtttaaaaagcataatataaacaatgttattaaattccaagatttacactgtaatctaatagagatgtattggtggtgttaaaacagcaattaaaagaaatagctccctagccttgaaaaaataatatgcatctttctctccatctcccaatctgatcattagcttgtaattgaagtaaatttcataaaataccaagtagttgactttgggatggcatttctatcaatttacttgtatccattatttttctgaaatagagaaggttagtagcaatatcaaggaaggtggactgtgatttatagagaagtttgcaattatgtgactaagtgcttaatttagggatctcaaaagtataaatttacaaagaaagttgatcagttgtgaagataattcaggaaatagtccagtaaatgaaattgcccatgtagtatcatgactaaataggggttttttgactaattctgggtgaattataattatttttataagttcattttaaagacctaccatttaaagacaaccactcttaactttgggtatatattttttccagcctcttgaaaatatattcatttattttggctatgtgtgtgtgcgcacacgtgtaccacacatttatatttgctgtcatagtatagacacgattttttatcttttcacctgattttctattataagcattttccatattattacagtctttatgaacataatttaagtaacgtcaaataaggcataccaaaacctacttaactaataccagactattggacgttatgtattatgtgtgtgtgttgttattataaatgacagtgcactaaagatattcagaaataattactttttcccatatttggtattcttccttaggattgactcataaggtaataattcctgattttaaaatatggacagtttaatgtttttgacagatactgccaaattgtttttctcaagtactttaccaattactcttccagccagctttgttttatcacactgttgggatcacttaatagcatcctttgctttatcaatctttttcaaattgagagtgaatgtggtattctaacttgggaggtgaaaaatggttatttttcatttttaattgctggcaaagtcaaatatttttcttgtgtctcttattcaattatattttctggggaggttatttttatttcatttttttgacttgtggttagaatatggggtggaatccattcttctttctgaatgaaccagtatttgtttatgtttctgaactgggtaggtaactcataaaagaaatgttttagccaagctgttgagttgcattctctgcctttaagagcctttatgcccttccggtgcatgtattcagtgagtgtcccaactacttccagtgtacagatttcacacccaggtgtatggccaatagccacagggtgagtcctgatactgcaattaaagtggcctaatccaataagtagacttccttgaacatattttctgtgtggtattagtgtatgtaaaatttgtgatgtaattctactgctttcacaagcctttagtgaaactcagtggattcaaaactcacttttcctaagatgactcccaaatctctatattttcagctgagttaacaaatgtgaaaataaataaatgtttattggctttgaatttgggtcagttaagagagacaaggaattggggaagcatgagataacagagggacatagtaagacatagcactaagaatttacatggagaaccccacaaaaatacaatacagggtaaaggaaataaagactcatagaatcaaacacaaatccagagggacaaagaagcacagaagaacataatatcattgcataattttctgggtttagaattttgtcactaaagacatataaaatgttgtaattttgcaactgtgggtgtaaggggtgacattgccattttgagttggcaaaggatttacttctttgttcaggaggaatttgaaaagtagcacgggtttctcaggtctggattatacctctcttcaacatgacggaattggccgttcctgttacaggaggctttacctttcaacttgggttgctgactcatttgacaattttggaccatgcccacagcttgagagtacagagagtttgttcaaagtacttaaaaatagacacacacacacacacacacacacacacacgtttcagctggagcataatgctaaaatacatttaaaatgtaagaaatttctgtaagtagctagtacagcattgaataggtatctttcttttcaataatctaacagtgcaggcctagaatttaaataccccagaggaattaataattaacaaagcccttaaaataactctttaaaatttcaggtgcttacatgacattcagcaggggaagcattttagttttctgacaagtgcccaaaatggtgttactgatgaaaggagactgtagattttagacatgaggcagataagctatggagctaacattatgctattgatatttgggggtctgttttgaatccttgtccaggtggaaaactacccttctgcactggtactttaaattttttccttgacaaaattttgtattaaatttgtagttaaagaaacatttggaacagaaaatttgggactaaaaattttggaggataactgtgatcaaacggtcaccttgacattaaaatacgtttttgatacatcaggttttgaggaggaatgcattctgatggccgcactagcgttagttctttgcaaaatgagttgctcttcatccttctgaggtgaattaattgactcgtctgaattctttcctgccagcaacaaatatttgttgaggatggctacatgccagatattctcccgggtgctagggataaagcaggaaataacacacgcaagatctctgctttcacagagcttattgtctagttggtggaggggcagtcacataataaattaccaaatggaccaacaaaataaatacttagctacctacaaagtactgctagtgataagttaatcgatgaaaagtaaaataggatgcagtaatgaagcagagtcaggaaatacctcttccttagagagaacattcaaactgagatctgcgatcctgaacatgtaactatcagggaggtgagcattacagaatgtgggaacagttactgtaaatcccctatggtgggaacaacccttgcattttcaaggaacagaaagaaaaacaatgtggctgtagtagaatgagcaaggggtggtaggaaagacaactaagcaagagtgaggtcatatggggccctgtaaggtaagttacagggtgggactcctgtttgcaatggaagtcattagaagatttgaaatacagaagtgtaatgagttggattttgttttgaaagataccctgagatgtgtaatttgatatcttagaaaggcaagaattgaaggagttgcaggcttttgcagtagtccccaaaaaagacgatattgtcttagaccaagatggtattagtaagaatgctgagaaatggttgtattcaggtgacactgacttgctgatgtattgactggaggccagagtggtcaggaagaaaaagaatcaaggacaattcctggattttggcctgaaaaactgggtgaattgtggtaacattattgagatggaaatgactagagaggaactgatttgggaaaggaaacttaaaagctctgtttgggacatgttatatttgacatgattattacatagaggaaggcacaattaagtaggcagtttacatatcaagtctgaagtttcaaggctatggaactggttgagatcacctgtgaataattgaaaaaagaagaggctcaaaagtggagtcctgggactctccaatgtttagaggttgggaagagaagaatccagcaaaggtatttaagaagcagcaatgagttagagaagaaacccatgaaagcctgtggttcagaaacaagtgaagacagtgagtcaagagggaaggcatgaccaaatactgctaagagaacaagtcatttaaggacaaaggtgtgcccaccagatttggcaatatgaaaatcactgacatctttgacaagagcagtctcagtgaaatagtagagatgaaagtctgactggagtgagttggggaaatagagatggggaaatagatgcaatgtgtatagattattatttgaagaagtgctatgaagggattcaaagggaaagggaggtatttgaccacatattttttgaagatggaagataccagaacatgctcatgtgctcatggtaatgatccaggacagaagaagaaattgatgatgtaggagagaaaatatatgattagaggatcgaagccctgatagggatggaatctaaaaactgcatggaggattggcttccttaaagaaataacacttcatttaagtcataggaggtaaaacttcacatacaggcaaaggtgaaggtgtgtgtataggcgggttgattatggaaagatgaacaagttcttttactttctccataaaaatgaggcatgatcatcagctgaagagggatggaggtcggatggtgtcatgtaggaagtttaagaagaaaagctataaagcagccattttgtacaatggaaaattaaaaactattgctcaaaaatatgattcatttaattgtaggaaggcatctgtcaaatacggtggccttaatttcagaaaagagatgttaaagtattctttctgatgatgattaagcaaaagatactgctcagattgctccaggtttatgataaaaatgttatcgacagaaaaaaaacacctggatttgtttttgatttggggcgactgagcagatatcctaaagtgaatggggaaactagatctcagccacaggcacccctgtaataatttgcccaaccagcaataggtattttgtttttctctaaatctttgcactagtggtaatttttgtatgccaggtcttcttctgatacttgaccctgacaactgcattcagggcgtctcactgagatctatctagaatgattctttttttaagtgtaaattatctcaaagggattgaacctaatgaaggtataagtaatttcatctgagttccatttgaggccttgtcttcacaaacattgccagcttgttttggcttttgttaaatcgttttatcaaaccacgagctgcgttttggccagacatggaaaggtttcaacctatctccaatctgttggtatgaaataacaggaaaagcctctttccaaaaataatctgagtgaaaagttaaaaattatggagctccccaaagattcttgcgcatttagatgcaaactctgcctcagtctgccttctcctagcctgccatggtatcctccttcttatgggtgatctagtaagggataaagtatttactgctgtggaaaatccacactagggagtcctaacacaccctggggcctggttagggcaaattctctcgaggaggtgacacttgaactgattttgggggatgaggtggaattacatgaaatctcagcagaacgaaggcatggaaacactaaacagcgcagagtgtgagaagaaccacaatgaggggaaaggagttcagtgttgccagagtataggatgtggagcagaaggaaagaaggctagagaggttggcagagggcaggtcttgctaggtattgcagggtattatgggtaagatgggatatggaacctgaaagactgaagcatgaagcccaggatttaggtttgagctcctagcccaatgactgggcccaagtgataaggcagaaggaaacctgggaaaatgagtaggatttgatcatgtattggttcaggtttgtcaatgagccctacattgtaaatatgcttcacatacaggagggaggaatttcctcagtgggttgacagaaagccctgttggggaataggaagagcctccatctttggagccatgcaggcagctgacttgaatctgcgagggctcaggaaaatggtgtctgtctttgctgaagccacattcctattaatggaatgaggcctagatggtagcttagatcagaggttctaaattggtagcccatggaccaaatctctcacaagttggggctggctcgccagtgttttaaaatttgattttagtgtttttattcagctctccaaagcccttgctgttggctattgttttacacttgcccatctcacactttacctactattctattcagctccctgggacttttgggtttccaagtcctaacttagaatgaaaaatgaagacgaaatcttgccagaacctcaatatctctgactccgagacaagtccaggcaacgtaacttccagaagctagcactcgggaggtgggaggtggaagttgttttcagagcagcaagaaattggggaggaaattctttgcagccatattggcagggtctttcctttctcaggaaggcagaggccagggtgggatggaccgcaggactccaggaaagtgctttggggatgttagccttgctgcaagatttaattttatgtggagatgatcacagaataggtagtttgtggccaggagcagtggctcatgcctgtcatcccagcactttgggaggttgaggtgggcagatcatctgaggccgggagtttaagaccagcctgaccaacatgaagaaaccccatctctactaaaaatacaaaattagccaggcgtggtggtgcatgccggtaattccagctacttgggaggctgagacaggagaatggcttgaacccgggaggtagaggttgcggtgagctgagattgcgccattgcactccagcctgggcaacaagagcgaaactccatctctctctctctctctctctctctctctctcttcttctctctctctctctctctctctctctctctctctctctctctctctctatatatatatatatatatatatatatatatatttaaagaataggtagtttgtgttgaggggctggaggaggatttctagtcaatggtgtttgtgatgggatgctagcggtgtagaaaggccctggatccaatgcttttaccttaaatgaaaaaaaaaaaaattaaattgtagttaaatggaacaagagaaaataatgtgaaagtacagttgacccttgaacaatacaggcttgaactgctcgggtccacttacatgtggattttctctgtctctgtcacccttggggcagcaaggccagctcctcctcttcttcctcctcctcaacctactcaacatgaagacaacaatgatgaagcctttttgatgatccacttccacttaatgaatagtaaatatattttcgcttccctgtgatttccttagtaacattttcttttctctagcttactttattgtaagaatgcagtatataatacatatatcatacaaagtatgtgttaatggactgtctatgttatcagtaagactaacggtaggctaacagtaattgagttttgggagagccaaaagttatacatggatttttgactgtacaggtggttggtgtccctaacccttgtgttgttcaagcgtcaactatagatataagcagaaggtaaaatctactataattgaatttttaaaacactaggatttcagcaggttcttttatcagaattaaaatagttgaggggccaggtgtggtggctcatgcctgtaatcccagcactttgggaggccaaggcaggcggatcgccagaggtcaggagttcgagatcagcctggccaacgtggcaaaaccctgtctctactaaaaatacaaaaattagccggtcatggtggcgtgtacctgtaatcccagctactcaggaggctgaggcaggagaattgcttgaacccaggagacggagattgcagtgagctgagatggtgtcactgcactccagcctgggagacagagcaagactccatctccaaagaaaaaaaaagttgaacgctgcttaaaaaatcatgtagagttttggggttttttttgttttatatttattttttatttttgctttttcaagggcaaattcctgaatgctggggggagatgctgtttctccatggtgatggaagacatgttttgtctcttcagatttaggctgctgccagagacaccgactgtagactaaagcagggagaattagctccaaagcactgggacagaggccatctgcttgtgaaagcagcttctaagaaaacatacctgttcccctatcccttcctgctccttcccacaggtcacttgccttaatggtgtttgccaagagagccatacctttgccttttctcattgcatttgtttatctgtttcaaattctgtatgcaaggcccattctaattgagtcaataaaataaaattctctaggagtctggttgttgtgttatgacttccaagagtccttgtttttgttctctaactacagttatgtattgtaatacctttatgttgtctctctattttagcaggaagggtgccactcaatccccagtgacagatgaagaagcagttgtagcttctgcattgctgtttcaatgatacctttagctctggataatgcccctggttatgtatgttgctcacagcttcagtgcacatacacacatacacacacacacacacacacacacgtatatgctagacactgagcatgagtctgtgccctcctatgtgggtcaaagtctatacactgttaggatgggactgtacagttttaatatgagtctttcgggttaggctttaagaaaagaagaagaatctgcttggcttgtgattattgaagccaatgtttttaatgccagaactgattcttctaccacttgtgacttctgtttgaaagttgctattaaggtcttaaggaaaggattttcccacacacatgtttctgaataacctattctggtcaagttcacagtcttgacctgccaccatgtttcatcctacctggtctgggtgcccagagacctggagcatctgagctggcaggatggaacttcttgtgcctgggcgtgccaaaacttttccttgacactgagaaagacaatgaggctctgaagccagaaaatgtctcggtgagttgaatagttacataaatgtcattgacaatcattgaattttaaagtagagttgtacacttcaaaaatgctacagaatttgtatgaagcataggacttgtataatcttggcaatggctgattttttgatgcgaagttcaggaagctttatttctcacttaagttctagattattcacatcccctcattattatttactgctctgtgttgaatggagaaaggcctctcctttattgtgttgcttacagctccaaagctggaacttagatttcattttattttactttaagttctgggatgcatgtgcagaacatgcaggtttgttacataggtatacatatgccatggtggcttgctgcacctatcaacctgtcatctaggttttaagccctgcatgcgttagatatttgtcctgaagctctccctcccatttcccccacccccttacaggccccggtgtgtgatgtttccctccctgtgtccatgtgttctcattgttcaactcccacttatgaataagaacatgtggtgtttgtttttctgttcctgtgttagtttgctgagaatgatggcttccagcttcatccacgttcctgcaaaggacattaactcattgtttttatggctgcacagtattccatggtgtatatgtgccacatgttctttatccaatctatcagtgatgggcatttgggttagaactgagattattaagctttgtcactatgaggctcacccaactgcttacttaacatctgtttgggctaatgccccatttcccagttccaacaggtcactcgaaatagtgcttctgctaggaactccctctctgctctcttaccctctcccaacttctcagcactactgacaacataagaaaaaccattctggagtggctacccagggttttcatcaccatgttatccccaaataagcccaaataagtttaattaacaatgaagttagttagtacagaagataacatttcccatgtatattagttggctagggctgctgtgacaaaattccacaccctgggtggcttatgacaacagaaatgtattgtcatatggttctggaggctggaagcccaagatcaaagtgtttgcagagttggttccttctagggatgtgagggagaatctgtgccatgcctctcccttagtgtctggtggtttgctggcgatctttagtgcctcttggcttatagaggcatcactctatctctgccttcattttttcatggagttctccctatgtgcatgtctctgtttccaaatttcctccttttacaaggacaccagtgaggttggtctagggcccacaatactgacctcattttaacttgattacctctgtaaagactatctccatataaggtcacattctgaggtcctagggggttggaacttcaacatatgaattttgaggcatactcaattcatttcacaacaccatgctacccaaatttactcatctggccatcttccagctcctcagaggtggcagcacactttcccttcctccttgctctagctgagggcattgcccccgggcctatctttggtgtaccttttcctgggtgatcctgccagactgcatggccagaaaaaaaacaggggaactttccctgtccttttccttctcatttcatcgttttcttttcttttttttttttttttttttttgagacggactctcgctctgtcgcccaggctggagtgcagtggtgcgatctcggctcattgcaacctccgcctcccgggttcacgccattctcctgcctcagcctcccgagcagctgggaccacaggcacttgccaccacgcctggctaattttttgtatttttagtagagatggggtttcacatcgtgatccgcccgcctcggcctcctaaagtgctggggttacaggcgtgagccaccgcgcctggcccatcattttctacttttctgtaacttggctgtaccaaatgcacttctgacctccccaggaagctccctttccaaatatctgtagttaacctcttccttgccttcatggtgcctcttctgttaggctttgttcttttctagaggcacatcatgttttggatatcactctaaggaacccaccaccagttttagccacattgaccaaattgaccagttgctttaggtatgtttttgaaaaaatataaggagaactttccgccctcaagagaatcacttttgtcccctgttgcccaataagttattaaagactaagaaattatataaatggtatatagtatctttatggaattatgtgatacattaacttggggctctgaacaagtccagcggaatagaaaccagtttaacttttttccagaattctcttactatgaaatttttcaaagaattatacagtcaacactcatataccaaccaactagactccacaattaatgtttttgctatatttgctttattccagtatatccaactatttatccctctctccatctatcaatctctcttgatttttgatgcatttcaaagtaagttacagacatcatgacatttcatccctaattatcttagcacatctattcctaaacagctttgtttaaatcagcatttccttatcgtatatgaacacaaataaaacacatatttttattcacatctattggtgacacccaaattttaagctccacagggcagactttgggctagatgctttggggtcataaagatactacctctgtaatgaaatctcagtttatgtgacattgccaccctgtctcatttgggttgatcacagactgaaaggggcctaatttaatcaccttattttatagatggggaaagtgagtcccagaaaggtggggactcttgtctgaggttatgcagccaggaggtggccttttgggcataaagctttttctactgaagggcaaagacctggcttcttcttgaccaggtggtgttttcatttggttctggtccttgcacactgctgactaccttagtctttgtttcacaggttcttgttggggcagactcactaggctcctagaagatggaagcagggccaggctttggcatcactgaatgactcctttgtaattttatttcttccaatcactgattacatcacactcagacttcttttccttggcacctcccacatgttgtcctctttttctagatttcctaatctgtcttctcctttctggtgaaaggggatgttttcctggagacgtagtcagcatactctatagcagacttctaaccctcttcataacatttgtaacacccatcacaaaatgggatctggggagggggtcacccaaagcagaaatggtagctcttcagttttatattcttccttaaagatgcttgtgattctaaaaattgtgttggtaatccgtaggagggctactatcatagtagtgaaatatttcatcctcagatccccatcaaagaaatgatcatggtattttagaataactgagggagtacaattgcttaaggaaatggataccccatttacctcaatgtgattattacacattgtatgcctgtgtcagaatatttcatgtgccccataagtacatccacctactatgtacccataaaaattaaaaataaaaaaggaaatgatcatggcatcatataattatcttctatacttaaaaaaaaatttcttgagagtatgtttatgcatacacacttcctctaattcccagaaggatttgaggcaggtaaattaaaagtttaattttatttaacagtttttataatgaataatatagcacacaaacccgagaaagacaaagctataatttctgggtttgattcctttattcatgggagactatgttgagataaagcaaaaacaaattttgtcttccacgattacaatacataaaagatagtcaactcctttcaaacaacaaagggtagagacaaaagcttggttattaaacaagactcattatgattgctgacattttagaaaatgcaatcatttgcatataaactgtgatgaagagacaatttttatggttttagacatattctgaaagaccttggaaggcaatctcattctagtatctcaaagcggctgcatctggagaaaggtttctatggcaacttatgaaagcttgatgttttttatctttttcaagagcataaatcatcccacagcctgaggcttcagtaaaggtctccattattttacaagctattgccatttgttttcatgttatatattttgattgtcttagaggaaagagagcaaaggttatcatgtttccgagaaggcttggagtctattttctctttttttcattttgtgggacaagacatgaataacatcattctaaacattgcttctcaatgatcaaaatgatggtacacattgcaatatttggtttatgtcacgtgttgtttagattttccccaaaattgtgactggtgcattctcaggaagacaagccagtttgaacttaaggaggaggaactatttggccaaaacacctcctaatatgtagttcagtagagatgccctggagaatgctgcactgttccacatgcctgcaaatattcctctaatgatacagtcccaaggctttggacattgatagactccaggtgatttttatcaacatattctttccaagaaagttaatttaaaaattctgattttaaaactctgcatgtttcaagaattttgttttagcaacatggatctctgtatgttataggaggtaataaggctgaggcaacacccattaagacaaagaaacagaaccaggtttcagacctagctctgccattgctaggtgtataactgtgagcaaacccttgaatctcttcgaacctccttttactaatccgaaaaataggagtaacggtgccagattcatggcattattgttaaggattgaatgcgtgtgagtgctgggaactgtgcaatgctgtacaaatgtaaggtggttattactgttggctgactgtctttctttccctttgaaaaagtcaaaagtttatgttaccatttctggatgaccagaggaaatcagtttcagtatgtcttaagtattttagtttcttatactgtatttaaaatacttatacagacactgatcactacagccatttatttatttatttactcagtaatcaaatgtcacccctgtagaagggtattaaataaattcattcaacaaacatttaagtgccaactgtgtactagcattgaggagacaaagaatagacaattaaattcttattgttcaggaaataaaagttttctgagcttcaaggccacagcataagctgttcaggtggtgccctgcccaagggcattcggctgatgaagtagaagggggatgtaatgcagtcccccactctgccagccaagccgtttgcatgcaccttgtgagctgcattcgcctgaatgaaggacatgttttggaaatttactagccaggagtgtgtgccttcttgcaatttacacgaaggcatgcatgaatgtgctagcagtggccctgatgcttgtatgatccgtgatgttaaagggaagatttgcaatgtttcactgtgaaatatgatgaaggctgctggcgtgcttgttatctggagtcagattgcctgaatttgaatactggctctgctacttgctagctgtgtgacctttgtgcacattacttggcctctctatgcttcattttctacatctgcctgcctcatagttattgggaggataaataagttcttaaaacacatagaatagcagctggcacacggtcaatgctcaaaatgttagctgttttcagtgatggctttactgttcagggtctccttgctactctgtgttgaaaagttcaacaattaacatctaaattctacctacaaaaaccacttttcttttatgaatttgatgtcaaattggtgatatttatctccttacctcagatctttttggtgtgtgtttgtgttaaataactagaaagtattctcttcagagaaatcagagaattccagttatttgatgagaagatgacttggtagtttttagaattttctcataaaaccactgctttgtcagagtgatagaggtgatgagggatgtttgcatattattggcttttataatcccagcactttgggaggccgaggcaggcagatcacctgaggtcaggtgttcgagaccaggctggccaacatggtgaaaccccatctctacaaaaagtacaaaacttagccgggcgtagtggtgcttgcgtgtaatcccagctacttggggaggctgaggcaggagaatcacttgaactcaggaggcagaggttgcagtgagccaagattgcgccactgcactccagcctgggtgacagagtgagacttcgtctcaacaaaacaaaacaaaactaaaacaaacaaacaaaaatgacaacaacaacataaaaaaaaaaacagtcccaagggaatgcctatatagtttaccaggattacaatagggattctttgaggtatagtgaatttcattgtcaattttggttaacatgattccctctctctcttttcataactttaaactgggaaagagtccttatgtagtattttcaagactattaactttgcattttaattttttaaaaaagttttgttaaatatcaaattttgatatgaagagtgtgaaacagattgacaaagccaagcatgaggcaggtggtgattttgattttacccctccctttgtattctggctcctctaactgcccttaagacactgtaaagagggcacttctgtgttactgccactgtgtatttcccagtctcccacagcatctaacttgggccattttcttggcaaaaaactaaaagtgcagaatgctaatcatgttgtacatcactgatttctaagtatttaaaaaatttgggtgtctactcgtaattgagattgtcatcacttttatgaaaccttttccaagtaaacttctcagaagagagatgcaatatttttataatttcataacatcaaatattagtctaccattatttgtgtgtgctgtgctatgattattcatccaagggcctgtcatggggacatagggactgcttctgaaagtgccaaattaccatttggttgtgagattataattgatactgcatgttaaattcaagtgtcattagctttttaaaaagatgaagtgatgataagcttgctcctaaattgtttgcaaaggttaaatatctaagagaaaagctggtatttaagattcttatatttagtcagatagtagaatgttttaagacactttatatcaatcagtgtatatgtagagttactgtgtttttaattttttgttttttgtccaagggtagtggctaagagttcaggttttgggttgaactctgactctgccacttactaattgcgtaacctacagttaagtcactgaatgtctctaagctgccattttttctttttaaaatgaggataataatattcctcagcattgtggtaaggatcagttgagctttttgtgtaaagcgcttcacccagaccaaagtgcttcatgagttatgatggtggctgttattactctgggcattttattttattttatttttttaagacagagtctcactctgtcacccaggctggagtgcagtggcatggtcttggctcactgcaacctccgcctcccagattcaagtaattctccctgcctcagcctaccgagtagttgggattacaggtgcccgccaccacacccgggtaattttcgtatttttagtagagacggggtttccccatgttggccaggctggtcttgaactcctgacctcaggtgatctgcctgcctcggcttcccaaagtgctgggattacaggcgtaagccaccgtgcctggccagtattttcatttttaacaaacaaattgttaattgcattatatcaggagattattgcataagtgtttaaacagtggcgattacattgtctaatgttttaaggcaaatgtatttctgctactgtatgatttttttttgcaatagtattgcactcaaaaattttcatacttcccagaggatataccatctctcatatttttgtttctatggcaaaatgtattaaaagttccaaacaaccaacatagaaaagaactcttgggaaataactgtctttaggtgagggatgctctgtagagttcattgtttgcttagtccttgagcagtcaaactattagtccttttatcagtcatcattgagggaggtttttgagctacctcttctagacaatcttaatcacctcttgaccagactccaactcagtttcctatgtaccctaaaattccctccttctaaattgcagtgacttccctaagccactgatatttggaccaatttttttttcagatcaatttctgtcaattgatttccaacaagcctcttgactaccccctatgaacattagtgagctaaattgtaagttacttccagcaacatatttttgtgttgccctttttaaagatatttttgtaattttctgtttataattgtttaaggtacatgagcatagagaactccgttcaatgatttgataagtcttttgtttgttttaataactgtttatatttaacatcagatattattgggtaaatgcatttactaaaagacggtaccttttgtggaatataaaatgctagtgtatacaagtaacgatgtatttccttctgaactcttttgtttaagcctcagcatgctcaagcggtttatctaaattcagtgataatagctgttactatggctgcatgttatttcatttgttgaattgatgcttggtaagaaaaatgtcattgaattgtttgcaattttgaatttaaatagaagtggttctttttccttatggaggtaaaattaggaaactggggttataaatcctgtgccctgtattcctaaatcagggttgtgcaatgcttgtgtgcactgcatggggttcatggactttggaactgttatcccatcagcaactggaagcattggctctgcccccggtgacagggatgggaagatggattaactcaaataatgaaatgtcaaatcagcctctctataaaatgggaattcctcctttaagatcactgatagacggtgactaaagccttggcttttcattatggtttttaatgtgggctcatattttatgttatatggattcttataaaccacaacatataagtgtgtcttaaaaacaagctgatccaaaaaagtgagaaatatcttttgaagtgtaatttctctttgtagcaaaaattggaagatgcaatcaatgaagaggatggccatgggggtccggggaagacagtgttgtataatggctgtgaatacagatgctgcagttaaactggctttgtcacctactccttatgcgaccttggtcatctctttgggcttcgattttctcggccataaaatgggaatgtcaacagtacttatctcatggggtcgtagaagttcattgaattaatttattaaaacacttagaacccagtataataagagtattagctattttataggaatctttttaattttgcagtagtggtgtctaaaagtcacagaactattatttttgaaagacaagatagaagcggttttatttacgttgtaaggcatgagagcatcttggcatggccttaatatttggtctcataaagcaaatgaggaaggtaattggaactgagcacattcagcccactcatcatgggaagagcaccagatttctgttctctgagaaagcttgctaaattctgtaagagtgcttttaaaaaaaaatacagtattttaagagctttgaggtcaaaaactacatccaggatggattagtaccccaaactttatacatgtactccacactatgctttgtcctttgtcaaaatgtattgaactctgcattaatggatgtatcagtcagggttctccagaaagacagaaccagtaggatacatagaagaatacatttactgggggaattggctcccaccatcacacagatagaggagccccatgataggctgactgtgagctggagcatcagagaagctggcttagtctggaagcctcagaaccagggaagctaatggtgcagctcccagtccgaggccaaaagcccgagagcccaccggaggtcactggtgcaagtcccagagtccaaaacctggagtctgatgtccaaaggcaggaggagaacaagcatcccgctccagaagagagagtgagggcagagacagagagagtcccctcttctttcacctgtttgcccctgcagggccccagccgattggattggatggtgcccactacattgagagccggttttcctctcccagtctgccaactcccatgccagtttcttctggaaacaccctcacagggacacccagaaacaatgcttcacctgccatctaggtatcccaccatccagtcaagttgacacctaaaattaaccatcacaatgggtaaagtttattgcatgtacatttacctcagtaaagctgtgggtttttttaagagctaaattcatggtggtgagaatgtaataggcattcactaagtatttttgactaaattaataattaaattagtcatgaatggaattatttcattcttcagtgatgggtcatatcaggaaatccagatgcataaggggtcgaattttacctccttgattttgaaactttacgtcaacttctaaaagtccaactttaatagtaaatcccagttcctggcacacactttgaaggcccactgtccctcagtttaccagtttttcatatttaccctgagaatgaagtcagtgactggacttagtcctgtgtctgcaactcatatatttctcttgagcatggccttgtgttctcatttatgttatcagacatgcaatttagtcattaaaatagacattttgatatagtggcagaggatgtgtttaagatttgagaaatttactaaaaaatgaaatcccttttgtcgtttccagaaacatcagactctgggcctctattgacaaaccgtatccacttgtaagttgaatgtaacaataggcggtgcacgtgagccagcatggacttttctcattggctgttagcatgaggagcttgtctggcatccttgtatttgatcctgatgtcttactgtcttttctcccaggtatggcagcagccaaacttctgcatgactctggactgaatgtggttgttctggaagcccgggaccgtgtgggaggcaggacttacactcttagggtaaggcattaagaatccggaggacaaatgtgggactgaagctgagtttggggtttcatttttgtctttttccccaaaagtcttcaatttcatttgactctaagagggtgaaaataactctgaaacattcttcacagcctctctcccagtttgccttcctttcaattcttctgttcctttttgtcttttcatctcatgatatttggcctcatagagttaggattgagtaagagggaaatggacagatatgtgtgtgcctctgtgtgtgtgtgtgtgtgtgtgtgtgtgtgtgtgtgtgtgtgtgtgtgtgtgagacagagagagaaataggaagaaaaataacataattatatgtactttccactcctaacttcgatgcttccttcacaccaacacaatcattctaatcatacaaactaaacttttttggagagactttctcccatttttaaatttattttttaaattttattttaacaaatcataattgtattacatttatggagtataatgtgatgttttcaccatatgtatacaatgtggagtgattaaatcaagctaaattaacatattcagcacctcactttcttgacattttttgtggtgatacatttgaaatttactctgttattttgaaatgcacaatacattattattactacagttactgtgcaatggatttcaaaacttattcttcctgtctagctaaaattttgtacccttcctgtctagctaaaattttgtactcctcattccctcagttctcaccccccagcccctgataatattcattttgctctctacttctatgaattcaacgtgttttagattccacttataagtctttctgtgcctggcttatttcacttagcataatgtcctccaaattcatctatgttgtcccaaatgacatttctttatttttaaaggctgaatagtatttcattgtgtgtatataccaagtcttcctcatccatttatccactgatggacacttagggtgatttcatatcatggctactgtagataatgctgcaatgaacatgggtgtgcagatatctctttgacatattgacttcaattcttttggatatattcccaaaaatgggattgctgaattatgcggtagttctatttttagttttccatttttagttttctgaggaacctccatactgttttctgtaatagctgtactgatttacattcccaccaatagtgtacaagggttcccttttctcttcatccttgacaacactgattatttttcctctttttgataaaagccattttaacaggtgtgaggtgatatctcattttggttttaatttggatttccctaatgattagtggtgctgaactttttccatgaacctgttggccatttgcatgtcttcttttgagaagtgtctgttcagttcctttgcccattctttaaaaatctggttatttgtctcttgctattgagttgtttgagtttcttatataatttggatattaacctcttatcagatgtacggcttgcaaatatgtaaagaaaactatcattttattaattgttcttttgctgtgcaggagctttgtagtttgatgcaattccatttgtctgtttttgctttttttcctgatctttcagggccatatccaaaaaatcatttccctgactagtgtcatggagctttccccttgttttcttcaagtaattttgccgtttcaggtctcgtgtttaagtctttaatctatttagagttgattatttgtatatggtgtttgcatatggtataagataagggactacttttattcttctgcatgtggatagtccgtttttcctgcaccatttattgaatagactgtcctttccccattgtgtgttcttggaatcttcatcaaaactcaattgattgtaaatgtgtgggtttatttttgagctttctatcctgttctattggttggtgagtctgtttttatgtcagtaccatactgttttgattaaaattgcttcataatatattttgaagttgggtagtataacgccttcacctttgttctttttgtacaagattgttttggctagttgtagtcttctgtagttccatatgaatttaaggattgttttttctgtttctgtgaaaaataacattggcattttgatggggattgcactgaatctatggatcactttgggtagtatggacattttacattattaattctcccaatccatgaacatggatgtgtttttatttattcacataaactaaacttttacctgcctaattttccttcttgtttttgcttcagcttttatttttttaaaagaattatttaccaatttataaatacccttattttaattgctggttaattgtttcaattctgacactgttgcctaaaattaatgattttctatttaaacacagagtcaagcaaagcaagtttctctgcaaggaaatgccctacttccatacattcaagatctgaataatagatatagaagctacagagtattttcatttccagagagataagacatataaaattctgactcacagctcttcttttggaaggattcatcaatgatatatatctgacattttgtactcattcttttttttaaattatactttaagttctgggatacatgtgcaggggtgggatctgctgagctagatcacttggctccctggcttcagccccctttccaggggagtgaacggttctgtcccactggtgttccaggcaccacttggatatgaaaaaaaaaaaaaaaaaactcctgcagctagctcggtgtctgcccaaatggccgcccagttttgtgcttgaaacccagggccctggtggcataggaccgagggaatctcctggtctgcgggttgtgaagaccatgagaaaagcaaagtatctgggccagaatgcactgttcctcatggcacagtccctcacagcttcccttggctagggaagggagttccctaaccccttgcacttcccaggtaaggcgacaccccaccctgcttaggctcatcctctatgggctgcactcacagtctaaccagtcccagtgagatgaactgggtacctcagttggaaacgcagaaatcacctgccttctgtgttgatctcactgggaactgcagactggagctgttcctattcgaccatcttgccagccctctgtactcattctttactttgagtcatctcctttataattgaatttgtcctcagcaaatatctactgagtacctactatgaatcaggcacagtaatccccccaaaatggccttgctccacagactttacagtctctcagggggacaatgactgttgtaattgcctaattatagcttatcaaggaaaatgctacagtgagggtgggtgacagcttggagtggtgccataggaggcataagagggtaccttaccagtcttgagagccagagactcagagaagcctgaaagccttatctgttattgactgtgacatacaccgcctgacctagttatttgtgatttcacacaagccttcaaacttgatctaacccttgttgtctactggccattgtttttgccattatgtgttcctcaaatatctctttttacctttgtcgtatggcaaaatcttcacatacttccaggatctcatcccttcctactccaatcaaaagctacttgcctttcttctgtgttaataccacttacctgttccacacaaggacaattattatatgttgctttacaaggttttgcctgtgtacatcttatctctcccagttcttgaaatcttcatattccttgaaaaatacagcatataagagtgccttttacgtaaagaagctggtttagtacaattaggtgctgaatttttaaaaacatccttctttcatttatttgagaaaatttattggacaactgctataggagtttggaatactttagtgagtaaaacaaagatgccttgtgaaaattgcatttttgaagggtaagtgagtggaaagctagacaaaaaatacgcaaataaacaaaaacagaagagaaggaccatttctagtgtttctaactggtaggaacctggtttttcttagacatactcagaaataggaaacttttctactaattttttgttcaaagttcgcccctcagtcattggaaatgaaaccaattcaaaactacgtaaatatactattaaacataaaagcaatttcaaagtccaaattatgaccaaatattccctagtgctattttcaaatgtctggattaacaaatcacataagaagtgatcgttttctttcttgctttttctctagcattaggctcctcaacattcacctgaagtactgagtaaagagattcgtcaataattcacagctcacaaattcaaagcactaaaaaccaagccatgttatggtatattgtaaatgatgaggtttagaagctcttgcctattcagagttcaatcaattttgctttaaagattgatttaataactaagtcatgtgaatgaagtagagttgataacaaaatctagtttttcgtggatatacccttaagctgtatctataacttgtgaaatgtcgatttgcttatttcaggactgtcttttgttattttatacattttttacaaattttttttaattttttcctatgggaaaacagaaccaaaaggttaaatatgtggaccttggaggatcctatgttggaccaacccagaatcgtatcttgagattagccaaggagctaggattggagacctacaaagtgaatgaggttgagcgtctgatccaccatgtaaaggtaagatcaggccagactttgaaggatttgaaaacttctctatgatgtttccttacacaaattccagatcattctctcagagaatcttctatatctctggatgatgcaaatgtattttataatggtatttcagccactctgagattcattcactgttatcaaaggtgaattaggtgggaattctacctatttaggaaggttattgatgaagtggtatcttccatgtggtaaaatgtttaacaaaacccataaagaaaaaacatttgtgctttatttattaaatatctatttaaataccgggaagtcttttatgttatataaaaacctgtgcaaagtttttaaaatgctgccctagactgcacattgtaaagagtatttgcaatatgcctaatggaatattcttacattttatcattgtggcctatatatcagctaaagttattcttctttggagattgacatcaaagtggttcaagtcccagatcccgtcttttgcaaggaagcttcattgttctccccaagatttctgtgaatttactgagtttctcattcctgtgatcatttgtggctcatagttctggcttccatgatacctatgttcattcacatctcacggcctgtgactcttttcttctctttgcttatgccaacctgggttcacactcacctctttgtcctgatttttctcagaccgccacaagcatatgtgaaaagcaaacgtcactgaagtttgcttgggtttggtgggcgggggaaggctcttaaatttgcagaaatacaaacagattagaactgaatgttggacattcattctaataacctcttagatcaaagcatcccctgaggatttctcactggtcacatttctctgcagattccagtctcccaccatgctgctggtcctcagactctcttcacatctccctgctcctctgtttttccagcatcctcatcttggtccacaaagtcactcatgttctctgacaatcagacagtcacctaatctgggccccatccaggagtcccatggaagaactggcggaggttttcaatttcagtctttcctctctcatcttcacttgctcctgtgggtggaagtaagcagcacaggaacttattcctcactggtagaaaacatccccttagaagacagaagaaactagcaacggtcaattttgatttatataacaattttgacatcctcatattatttgtgagtgataatatcgaaacaaataactgaccataaatcatgaaacatttaataaaatgggaactaagcagttacttaatttggtataatgtgggtaaaagttttccttaatttataaataaatgttttggttgaccttcaaattttattttatattggccgggcacagtggctcacgcctgtaatccctgcactttgggaggctgaggcgggcggatcacctgaggtcaggagttccagaccagcctggccatcatggcgaaaccccgtctctactaaaaataccaaattttattttataagcctttccaccttccttccctatgtgtctaggagaaaaagagacacatgaattagaaatgaaaatctaccatggtgataatgtgatttgttgaacatcaatcaacagttcttaacaccctttgttgggttctttgtttttttaaatgtagattttcttgaccgatttcttatgtcttattctacctgtaaggcttgcagagattgacttttcagaacactaggatctttaaatttctccagacaaaggaaatgaccagagattatattcacttgcctgtctttgtgtgtgcagagattattgtcagctcagagctatgtccaggatgctttgttttttcctgacattaagtcccttgtctgagagaaattgctgagtcatcaattacaggaatgatgttacacttaaatgatatttcacagtgatggccaaatgtgctgctttttcactatttccattactctatgtgcagttaggaaaatacaagtagttaagcagtagtccttacttaatacagggtaaatacatatgccaataatgctctttatatttaaaataagtcttactgctttttaattatgacaaaagtaaagcatgtttattgtaaaaatatgattagaaaatatagataaactagaacaattaacaaaccctttataatactatcttgagaagatcactctaaaatactctcttggttcgtagattttcgtattcctgtattgctattttctgacctctgctggaggaaatgggaaataacagtgcattttaagaaattgtatgcacatgcatatgtgtatatgttttacgtagtaacttactctcaaattaattatcactaatgagacaaattgaaaaaatactgatgctgtaaaaaaaaggtttctgcagtcttgacaaaggtgccaatttggcctcctcgtgatcagtcacatgcagtgaagagctacatgataatacataatgacgaagaccttatagctaagaagtccttctcaaactaagtacttgttctctaccatctccacttccatgtctttgtatacgtcatttttctcatttttgacctgtaaaaagcatcttggatggctacattcatttccggaattattaacaagaacttcgacattctttctcctaccacatactagagaatgtagttgagaaatttgcctcctgtgtcatggaaagcagtactttgggaatttgaacactgccctctattacctattttaataactactgtccccaagggcaaactacagttcatgtaaatagatagtatatttgggccttgtttcttttttatcagggaacatgcatgtatttcttaatctgaatcttgagagtatcaagtatgctacttgccatattgtcagatcctgctatcaaagaatctgcttttaaaattttttatgtggctgataatgggaaatagagttttatgtgcaaccttagtaacattaagctaaggaacttggatatactggttgatattgaaatgaatgaagtggagctacccagaaaaggggaagggcacagtagctcatggtggactaactacccacatgaaagagtgtgtttcctcaagagaggatgactcccaatatcaccagttctgtggtagttgtcatagaaatgttcttctgatagaggaagtgtgttcatgccagctccataataggcatctttaaacacctagtgtgctgtgatgaacaggcctctgtcttgatctgatctgtcagacatgtttgtatctactgagtggcgttcatttttaatgctctgtagatctgttatatgttgttaaagtagggttttccaaagacaacttcataaataaaagatgtgataccaaactatattgggatttaattatcagtgagaaagggatcgcttcagctcaaatctatataatttagaaggtgttttccttacttctggagtcagtgatgcagctgttagtactttacaattattgttaaacatctactgagatttttgatccgttttacaaataggcatgctaatttccactggtatagtttagaaggcagctgtttagatgtcttggaagtaacttgaaaaaattgttttcttttaaggaatatttcataattaaaaagaaaaagataaaaacaaaaacttcttaaggaatcctgctatattttgacttatgtttctttctctttcattgtgtgtttacatgtgcatgcgtgtatggttgtctttgttcttttgggctctttgaagaagttggagaaaattctaaggtttggtacaatgtaggcaaataaaatttttctgtttcagaagctttcatcagtctgaaatttgaaagtaaagtctggtaaaacacccatgaaactgctctaggtctgaaggttgaactgttaagagttttgccactataaagatgtagtgtgacttaaaattaagagtccaacttcatactgatgttcatttccaaacttcagctatctggagaagctgagcaaaaggactttttggtcttaacctacttcccagtgggcagaaacaaagcttattgtcaaagtcctttttgcattgcatatggtcaaccttcaatgctaaagatgcatgcgaatgaggattcatctctcaaatatattgtctgcttgttgctgccatagctgctattgctcaaacagcctcacagaggaggaggcatttggcacaacccctcagtcttgctgacaactctgaaatccagttgaaaatatgatacacaaaatgcacacaaaggcagagaggggaaaccatagctatctatctgcgatgccatttcagttaatctctctgtctaaatggcctctcagtactaagaaacagcaacaggattagagtagaaatattgagacataaaaaatgcaaatgataattgcatttagcaaatggaaatcgtcctgttgtgtaaggtcttggcatctcctggaaatcaacaggccagaagtatccagtcttctctaggtcctcaatattcccttcttcacacccctgtccccgatcctattaatccaggggaggctggatcaaagtccagaatacacttgcttctctcataaagacagaagtctccaggaacaggttagaccaactcttgtttttattcaggaacagttgcccattttacatgaacttcacacttaccatgttgagtttactggctctgtgagtttgccctttctgaagtgggcttaatgaaccttttctaccacttccacccacactgcatttcatttcttatttgtttgaaacaaatatgtcttattatggaagattttttcaaggaaaaatgtggagaatagtaattttctctctagtaagtgaaacacatttgtctagtgatcattctaaagcttatgctgttattctggaaaccaaagtgctcatttgtgttctttagagaatacaggcagatctttggcatgtaataatttgctgaaaattatgcctttgatggctgaatttggaacaacatttaggatatgagatgaattcattttccgcctccaaggtttccatttggaacttaaaatatggtacaatcagtaaacatattttctatgcatacacacacatatctggataaacttaacagtgactatggttgtgggtaacagttagttttaaattttgctgggagtggagggtagacaatgtatggaattaagttatgatagtgaaattcactaagggaaacagcgatatagattaaatcttgtgcaaaattttacagcttctatactatgtgatcatgtgttatggccaagtagtccaaaggagctgcaaagacagggggcccagctcaccaaaagatggtgactaataagggaaccatgtaacagattaaagagagctttggcaacttgcagtaccaagagattgacagaaagtgcaagatggcctgaaatgtgttagcctgccttaccatgtcctctgcagagcagcagcctgcagaaaggcttaggcgtggattcccaggctgcgtatcacatgtcctgggcatttctcttggcctctgcaaccaccaagaagtaataacaatggtaacattactcttatatggacatctagaaactaccaagtgttttcaatctcaaataactataagttatttagttgtgaattagaagtattatccccatttaacaggtgaggacctaaaggttaaagagattaattgcaaatgacaagatgcaatggggtcagagcatgagttgaggcttttgggtgtcaagaacacactgcaaagagctcactctctgctggttggggactactttttgtcatttctttctaagcctcagcacccacctggcccgcctttcttcttgccaaacttatactctcacatattggaaaaatcgagttcaagatcctcctttccttaagattttccacagttgagtacagttattccactagctccctccaaagccctgtatcctcctcaccttcctgattattctttataaaagtctgtttttaagtaggataaacagttttctgttacttgtacatcgagacttcataaacagttgactcttggacaatgtggaggtcaggagtgctgaccccctgtgcagtcagaaattcttatataacttgactccccgaaaactactaatagcttgctgttaattatgttggtaaacacatattttgtgttaaatgtattatatgctgtattcttacaataaagtaagctagagaaaagaaaatgttattaagaaaatcataaggaagagacaatgtttttactattcgttaagaggaggtggatcatcataaaggtcttcatcctcatcatcttcacattgagtaggcagaagtagaggaggaagaggaaaagtcggtcttcctgtcttaggggtggcagaggcagaaaaaaatccatttggaagtgaacctatgcagttcaaacctgtgttgttcaggggtcaacgttttgtgtatgtgtgcaaaaaagcaaatgtattacaagtaaatgctaacaaccactgacattctaacagtttctcttagagctttaaggttggtaagtacttggttggccttccagattatccagatgattgtacttgatgaacaagtaaagctggcgacagttttacgaatgctttatcattttttctacctgtcagtcttgtggcacctgtttgctggctacatgcagcctgtccactaagacaaaggcacacacaattggaaattttgtcatagcagcattctagttcagaatatcaccaagtgataaatcaagaattcaggaatggatcagctttagtgaaactggtgttgaacataaaatatatctaaataaagatttaaacaattggaagaattacaatcatagtaatttatgtacatgttattaaaaatgtttatatggtaaaaattatataatcaacaaaatcagaatgtagagaaggtgagaaaggaagacacataagagaggtaacagctgcttaaatctttcatagcaatgaatcaatctataccaaaattaatagttaataaatagttaataaattaattagttccctcaggaactaatatctcttagggtgtgtgaaacatctatttgaagtttagcacttccttcagttcatttcagtttatgtttcttccatcaaattgaagtatatttccatcatttaaaataacagatataatatgattcaattctcatattttttattttctctttgttcttttctccctccttcctttcttccttccttgttttttgtttccttcctccctctctcagtcatccatttgttcatttatccatccatagcaaccatccatccattcgtctattcatttttctatcttgtagatgcttatataagaggtctggaatgtcatacaccaaatgttacggctttttttttgtttaacttgatggtacaacatggagtaattcgttgctttcttctttgtactttttagtactgccaaaacattttataaagagctcctctcatttttatttttaaaaatgtaattagacacagactttactttggaaagctcatgatctatgagaagaggttaggcccagtgtttctagcagatctctgtgcctctcacctgcctaggcagcagtctcctgggttacatatccattaacaatcaccaaactgcttccagccaggcttagtgactgagcttagatcctttgagttcagacagtctagatcccaaagcagctgttctaatgcagaacctcaaaggcccttatcctggtattattgtgctgcagaattttctgagtgtctgacacatacacacacacacacacacacacacacacacacacacacttaatcattgaccttttgtgtgtccttggccacgttatttatgcttttgtgttttgatatctctgttgaaaagaaggatgtttgtacctgtcccacttagtattctgaggtttaaagaaacaagatgttaacaagacactgattaacatcattgtcacgaggctgctgtgatacactgaagatcctaagaacattttgataggaaggatagagtttctttactttccttttggaaacaaacttttctaataggttctggggattcttagtagcaagtaagaatgtaaatgatgagacaccaggtaagatgaagctttacaaattcttttcaaaagaggaccaggccaataaacttacctgaaaatattttcatgggcttcttatacactgaactgtgaactttcccccttaaaatccagtattatttttcttctgtgttattggtaggctaggagagaagcatttggctgcaactaaactcacatgcccaaacaggctaaatcgatcataaatagataaataaagtgatcttttctggctgtattaccttctaagtttccttcagttccagtcagacttttaataccctagaataggggacaatggctattactgggcttagctgagatcctttcctctgggtccctaactggccatgctggcactcttgtagagtcaggaatgtctcctcctgtcaggagacaggaggcatctcaggatttactagtctctaagaaaacctaagtttagagaagtaaaatacattactttaaaaatctcttttgatatatgcgtgaaatctaaaagtattaaaatagcttacaacagcactgtccaatcaaaatttaatatgtacattgataattttacatttttctagtagccatattaaaaagtgaaaaagatgaaactaatttttataatacattttatttaacccagtatatccaaaatattatttaaacttgtaatcaatataaaacattattaatgagagattttacgttcttcttttgtactaagcttttaaaatctgatgtgtggtttccactcacagcatatctcaattcggaccaggcacacagtgctcaatagcctggtgagtggctactgtattggatagcacagggataaaaggttagtagattctgtgtatttttgcaaacattgctaatccatcttaaatttgttaaaaaataaaacccgtacaaaacatatgtctaaatctcacaacagagaccctacagtacatcgcaaattaacttcctttattctgttaacttcaaacatctgtcatcacaaagaatccagaagtaaacaatgagtgaagttccttatgtgcctgctacttcctaagggcagggaaactttgaatcactttgagaaaactatcctaggtacacagggagatgctatgtcctgtgattttaatgcattagaaagtgagcaagctggaagtaattgaggttgacgtggtcagagagactaccctaagagaatgctttgaacacttacaaaaaccttaaaagacactgcgcaataaattcaagggaataaatttatggagagcataaagacttttcatatagtgtcattattttaatacatttgctcatttgtccctgtctatgactaattcaggagaaacaatagaactgtcccaaagtgccataaatggtgattatcttaacatacagtcagagaaaagtccaacaagtaaagagttgtagagaagataagcctgtagttcaatggaagtttatttactcttttcatcttttagcacacatgcttcatgcaaaattctgagcaaaagaactgcagagcgacctggagcattttactgctgacatttactatttccccttttttaaagttggcaaatgttaagggcagttgctacagacagcttctactcatgtgcaaaccatgagaaaaatcacaattcatagttacctataatttaggctctcaagggaaaccaaattcatatgtacatggtggctcctggaaattctgttccaaactcaatttaataataacaataagcaacatcttttgagattttgatagatacaaagcaccattctaagcagtttatatgcattatctcacttaatactcagaaaagcctgatgatttttattatttctccttcacaaaggagagcattgaagtaagtacaaggcatttacacaacttgctcaagatgccccagttggtaagtgatggagtgggggctttaaccctgatccatctcactccaccatccaggtatttggcagctcagcttaggtgcaggccaacatagagattatacttaagagcagatgaagtctcaaaaaagacaaggaaaaggataagggtgctgaggactgaattgcggggcaggccctcaacccttctcccctttccgttcaggttcttgcttcctaatgctgatttttttttttgtcttatgcctcatcactgatttttctttttatctccatttgaccacctgtgacctacttgaccttccagtggaggacactgacatgaatcatctatttggttaaatcaaggactattgagagacattgaaatctctcatttcattcttaatccaggaatttaaaaaaaagtattaaagctgctcatttgagtgagaatgctggaactctgtgtcacacaagataaacgtaagaatagagagccatacatgtttcttgggtttatttcatgtttccattgcaaagtataaacataatagggttagaagaagcattgctttctgtataacttcatacttaggcagaaaggaaaatataaaattacatgtttaagggtgacctatgtggagtagatgttttggcaattgaaaggatgtcattatgatatctaataacattgatcctttggattagaaaggatgagagtccatctaaaaacaacaggttgtttttaagctgctacttttcttgatgaggccaggatagttgtgctgctgctattttagggacctcatatttcttcctgattggttccaggcatttctcccagatatctgttgacatcttgtctatgtatccaggctggagctaaggtttcttgactgtagaatcctgggagaaaaagcagtaaaaataaataagttagaaagatagtgaataaaattaaattttcatcatgacctccaagtacctaaatgatatgccccaccaatctcctggcccagctcaccctggtccagccactctggcttctagtgtgccaagtttattcctgcccctgggctattgtgcttcgaagcagattaaagatgggtggctacacattctttgatagtcttcccatggaaagggagagttggggtccatgcctcctctctatgaatctgggaggactctgtcacggctttgaccaggagaatatgactgaagttatgctactccagtttgacagcctaggccttaagaaactggtgggttccacttttgaaaccttgagttacaccatgtaagaagtccaaataccctgagactgccatactggagaagccacatgtaggcactctggtcccctgtgccagccaaatccaaccttccaaccctccttacaaaggtactagacttggaagtgaagctgtgtcagacatccaacccagttgagcctttgaatgactccagccccaaccgccatctgacacagccacataagtaaactccagcaagaaactgcccagctgagttcagtcaatccacacaactgtgagagaaaataatagagtgatgccttaagccattaaattgtggggttatgtttttatgcagccattggtaaccaaaacacacttgctattccctccacttgaaatgccctttcttgggcctcaactcaaatatcacctcctcagagatgccagagtagcctctcccacccccactggtattctctattcttaatttaggctttctctgctttattattttttatagcacttataaattatatcatgtatatcatattatacatgtatttgtttttgactactttctcctggtagaaggcaagttccatgacggcagatactttggttggaatatgtccccaaaatttatgtgttggcaacttaatccccagtgcaacagttttgagttgtgggacttttaagaggtgattaggtaataagggctctgctctcattaattgttgctgttattgcaggagtgggttagttaattgtgggagtgggtctgtcatcggagaagtggactcctcataaaaggatgagtttggcccctttccttctgctcatacttgtgatttctcaccatgtgatgccttccaccacgttatgatgccacaggaattccctcaccagatgccagcaccttgttcttggacttcccagcctccagaactatgagaaataaatttcttttctttataaattattcagtctgtggtattctaatacagcaatacaaaatggactaaggcaacaaaattatttctttttccattttgtccactgctgcatctccagcacttggctcaggatgtggcagttggtaggctttaggtaaatgttccttgtgtaaatgattgaaagaatgggtctttacccgtatgtgagcctgtcccttttagagcacaattgggcagaccctgatttggcatcactcttaggagaaaacggaaatattttagccacaagcactctagtcctacaggaaaagaagtgccacctagtatggtgtcaggaaaccaggagggtcccccacctcaacacttaacatcaccggctcccacccaaattccacaaataaagactattttctttgtccacagttgagttacagataaactggagatacagaagcaaacaaaacatacaaaaatccctgctcttgtggagcttatgtgttatctggggaggatataaacaaacaaataaaatatatagaaaaatattggtatgcctaaaataaaattagtcatgtttgattttataattgcttttcacttgcagtaacaggcacaatcaagaaatatggctaagtgcagaataaaaaaggctataaaacatggaccttcttaaatgaagttaattcagacgtaacaaaaattcatatattatgttccttgaaacttaaaaaaatgcgactttaaatttaacactctcaattctaatggggatatgagttaattttcaagtatattttagagctcaagtttagttaaccaataacttgctgaattatgcaaaaagctttggctttcaaaatcttattgcttttcccctgtcaagatttaataatttttagtaagggtttgaactttttaaccagatatgccaaatctcccaaatgcatgtataagatgttattatgttaatagcaatgtataatacaatatctgcacacattggaaaatatatatgtgtgttgtattagaaagtgatgagtgctatggagaacgggagtgtggggttatgtgagagggtgggatccaatttcaagtagggtagtcagggagggcctcactgaggaggtaacatttcaacagaaaacctaaagcaggtgagagagcaaaaaacttaaagtataataataataaataaataaattaaaaatgggtctttgggtaagagtgttccagccagaggaatgtgaggttcagaagccctgaagctgttttgtaaagcttacgtttacagcactgcaaggaaccccctgtggctggagtgaagtagacaaaagaaagctgggggagggaaacagtggttctcaaaaaacaaacaaacaaaaaacaaaactctcacctgtagattttgcacggtgtaaatacttaatgtccgatgtcaagctaccaacttaccgtccctgaaggcagagttggaaagaagtgaacacagatggttctcatgacacagtacgcacagactccaacacaatatgaggaggtcagagagagaacagggctaaatggcatagggcctagagggcaattctaagaacattgacatttactctgggtgatgtgggaagccactggaaggtttgaagtagagaagtaacatgatgtgactttcctttgtaaagtactattctgcagaacctccttcatgagcaaatagatgtgtgtgtgcatgtgtgcgtgtgtgtgcacatgtgtgcatgcgtgtgcatgtgtgtgtgcacgtgcacatggccacacatatgtctgtgtctatttcttcttcatggacggcaattcaccccagctgttactctgctttctttgggggcagatacaaaagaagaatacaaatcttttctttttttttttgagacagagtctcactctgttgcccaggctggagtgcaatggagtgatctcggctcactgcaacctctacctcccaggttcaagcaattctcctgcctcagcctcctgagtagctaggactacaggtgtctgccaccatgccaagctaatttttctatttttagtagagacgggttttgccatgttggccagactggtctcgaactcctgacctcaggtgatccacccgcctcggtttcccaaagtgctagaattacaggtgtgagccactgcacctggccacaaatcttttcctatgaagggccaaacctctttcttcatttaggcatttaacccagaacccactgaaataaaaatgacaatattaatcatgatttttagactatgtggctcactcaaccatagagcttctcatacaagtgaaatgcagcacatgtgtgaagccttaatatatcatcacaatctgttctattacttcatctcatcaattggtaattgaagtattcttaggatcctgctgtgttctctagctttgaaactcacagcatcctattcaaactcatgtacatatgtgtgagaaatgggagggctgtcagcagtcattcaataattttgaagaggagcacttcgaaactacacttagaccaacccgcagttgtcattatgacggtcattgctgaaacccactttaggtcagcatgagttagctagcaccttgtggcctgctttggaatttaaagccatcatatgagacaatatctctgaacagaattttaaaattgaagctatacataagaatggtatgggaagtagggaccttctgaattaaaagtttaattttgggtgggtccaaatggtacagatcaaagaaagagaaaatactagcacagtgaccgacttcctgagcacaaatacacaggcttgaagatggaaaaggtgaaataactgaacacaatgtcaagaaaaagaaagaggcagatgcttataaatgtaacagaagccatgaattattatataatgtatcctaaagaatttctctcctagctatgaaagaaacagcctttgcctcaggggtcttttgctaatatcttctagcagccccaagatatgtagacattgtcatatcaaagttcctcagagccttgaacaacatatgtgactgtgtattttcttgggaaagttgaaagctctaacaataaatgcatctgtaggcctggcgtggtggctcacacctgtaatcccagcactttgggaggcccaggcgggaggatcacctgaggtcaggagtttgagatcagcctggccaacatggtgaaaccccgtttctactaaaaatacaaaaattagccgggtgtggtggcacacacctgtaatcccaattacttgggaggctgaggcaggagaatcactggaacccgggaggtggatgttgcagtgagccaagatcatgccactgcactccagcctgggtgacagagtgagactccatctcaaaaaaaaaaaaaaaaaaaaaaaaagaccatctgttttagatactgagagcataggcttagaacccagaggggcctgggtttgaattctgaactcgctatttactagctgtgtgatttgaggcaagtttcttaacctctctgtgcctctgtttcttaatctaaaaaatgaaaataataataccttgcttatagggttgttgagggagataaataaaaataaacgtataaagtcttattaaaaggattttagtatgcagcaaatgtgaaaaaagtgttaaccatgatgatgatgatgatggtgatggtggtaatgatcatgatgatactggtggtggtggtggtgatgatggtgatggtgatgatggtaattatgatacttgcctatcacaatccttatttctcatacccactttctttgtgctcatgacttctcctttgaaatggcttttcaaaaagcatatgggtgtcaattcaaagtacccattaagtgaatttctttgaaaactttttcctcctgaaaataattgtttcaaataaacagatgcctctttgatattctttttatctcagtccagttggtaaagtttgaatgccctttaagtatctccagggtgtcttccatgtaaaattcacaagtagctttttggccaaacttgcctcttccttcatctgaatctcactccaggtttctcctgctgtgtcatctctcgactagtcttcagaatattcttctaatcagaatcttcccagcatccttcttattccctcaacaagtgaatctcctttaaatcaacacaatttctacactagggattaatgttcatagcaacagagctccttttgggaccaagaaaacctttctatttgtgcataaagtctcctttgatttattttaaagtggagttcttatttcaaagcattgactttctttggagaagtattctgactcatctaagtgaatcatcattttggcttgtatcactaaagaaagtgaacacttctcccaaacaatttatggagtgaaaatttggtacctgcaccagcattaatcagaggctgactttggtactggatgagttattcaatggagaagagaaaacatgttgtgcttggataaattcgaggatatgaatttctgtctcataaggctctctctgtagagaaagacaagctaattctggagacacagacttctgttacactcctggggcttcaataactttaccatggaccttgggcatgtaatttaatgcttcgtagaagcttcaattcctagtttgtaaagtgggattattaatttctaacctccaagtgttcccttgaaaattaaatatgataatatatgaaatgactttataaatatcaggtaccttcatcatttttaaaatcttatgtggtagagaacctctttagaaaggagttttttgacaatttgttttttagaaacaattttttctcaactgagataatcacatgtcctcagatttcaaaaggataatctaataatctgaggataataattgacatttaaggaagaacttgttttgagaaaaatcttttattttagaagtcaatttctccctccctctctatccccatccatccttgtatattgtactaaggcacgtacccaggttaccaagaacttttccatcttctcattactttatacatttcagaggcatcaaaagcattcggataatatttttgaaagacaaggggcgcgcctgtcatccggcacctgtgagcccagtgaggctgcagccgggataggagagtggtgcagttgttttggattagctgatctgctctctggggctggagttcagggtccagtcctggaggttcagagagggcttgctagaaaatgcaattaaacgagtaccttccatgacaaggaggtgctagggtaagcatttggggatggatttttgtgctggtaaatcccagcatgctcagtgatgctgtaaaggcgagaagctctgagctttcttctacaaagtcatctgctagttcatacggtagaattatcccagagggaggcaattgccctatgggaggctcaaggtgtgtgtagaaaggggctttgtggtatttattaaaatcataataacaacaacaactaatatccttctaagaactttgcatatatgatctcatttaatctttgccacagccctggaggtaggtattagtacctacattttacagatgatgaaagtgtcagagatgtaacttacctgaggtcatagaattagaatagtcatttcttgagccaatgctttcatcatctacatgaaagttggcaatactttttgtggaaagaaaagtgtagggatagtaaggatgatattagtcaatatctatgcatttactatgtgcaagtcactatgttgagatgtgtatgcattatatcactgatgacccataatactatcatggcattggttctattctatttacattcacattatatacagaggcccagtttgttgcatgcctgagttcatggttacctgctgggatgttgaacatcacaagctgtgctctcacctctggtatctaatatcatgtatctgtacgcaaaaacggactttttgcaagtggtttctggtgtttgaatgttataaaataagagtttgcgatgattatggtgaagctgagtgttcccttttttgtaaatgctattgtatttggttttatttctttgctgctgtacaatgaaatcaccataaaaatcactttatgtctgtagtgaaattttccaaaccataacatatctttatgaacctgaaattttacaattctttaataacagctatttaaacaagcacttttttaaatatttttgtctgtgaaaaaccacaatagatttattaattaaattagaatattagagctgggaaaccaccttctatgtaaattattggtgggagtttatgaaattcttgtagtaagactaaaagtagagtgatcttttctctaagaattgtacttaagctaatacagctgatagaacatgttaaaaatgcatggaagacaagatttcaatatttagacttgtttaagatttattggaatttggagatcaagtggactttaactccaaggtcctttcctaaataactcaaaatgtataataggagttgttgtttaggttggagacctttctaaaacaggaaattcacttttgttcatggcacaaacctttataaggacattaatggtgttttaaaattatgatctatgatgtaaaaataagctttgtcttgagggccttagttagatttgactacagactttcttctctcagtttggtctgttcacctatttgagtatgtttgtagcagctattgctctatgtctcatttcctttagcaaggttctgataagaataatagaaacaattgggaccttgccaccaatctccgccccaaaagaaaacacctcaattctcaaatgaggtcccattaagcctgtgtcagaagtttctcatgaggtctgggccaccccagagccctgggattgagattttttagacattgctacaggctgctgtgcccatttcaatggatggctgttgcagttgggttcctcaagacacagacttggaggtggcgaatagcatgttggtggtttgttagtgggtactgtggggatcaacagccattgattgttggaaggcaagaaggcaggggtggccagaggaataagtgtgatgtagttgcagtggaagcctcagctgacctgacaagggattctgaagatgagatggcccttgggagctgtcctgagtggggcaagagggccaggcctttctatcctcatgtagatagtcattggaagtgaggtgcccagagaaggtgacatgaccttaggcaaagtggattttctgcagctgggataatctctgaagggggctgaaaatcaagggctgcctgccaatagcactccgagtaactgaagtaataagttcctaatttctgaagggcaatctgtgcaagctcatcacagcatctgccacattgaccacttgggaactccactcttctctttagtagttccacgccaaactttgtttattggggcttttgcggaccttgccacctggatgacccaaaggctctggacagagaagcgtaagagtgtctggtgagatcaatagagtcatgaatcctgctgactacactttccatgaaacaacttcctttatccaaagactagggttgccatcaaggggctgttccatacacagccacatagccaggcgaagctatgaagccagccatatgccatgttataattatgatgccgtaaatctctgttttcatggacctgcctctccaggactttggagcttctggagcctggaactatgtcttatttaatttccgcttcttcagtgtatttcttaatgcctgtttcatagcttgcgctttttccattttgtttaagtgttagtagcacttaaaagtatgatgcctagatttctcctgggtctgtccgagcctgtcagtagttttgattgtcttcatcagttacccaaatacagtgttagttctaatttggtagttatcctttgcgttgtcgctctgcctaatactcttaaagtcacaattatattgaagtagagtagaatggtgatgaggtgggcaatgttggtgcctgctgttgcctgtgtgcaaggatccatccaggacttggatcttctgctgcatgagaggaagcaggagctgggaaactagcttgatgttaagcacacctgaatttgaactctgcttatcagctgtgtaatcctggcgaagatgtttatcctaagactcattctcctcatctgtaatatgagttactacacaaatattcaaaaagcaacattattcataatagccaaaaagtggaaacaacccaactgtgtatcaacagatgaatggataaacaaaatatagtatatccatatataggagtattattcagccctaaaaaggaatgaaattctgacacatgctacaacatgggtgaacgttgaagatatgctaagtgaaataaatcagacacaaaaagacagatattgtatgactttgtttatatgagcattattactatgtgctctgaatctcttctggccactaaacatggtttcaaatgaacacactatcagatatttatttattcttcaaagatttattgaatgagtactcctccaggtactgggaatacaccagtgaaaaagacaagatttctaccttcgtggggattacattccagcgtggagaggcactcaatatatgtatatatatatgaacaaatgtaccacatagtctcagttgctatgaagaataataaaggttgacgggaaaagcatctctgaggaagtgacatttaaatagtgccttgtgaatatctggcagataaatattgttgaaagagggagtgacaggtgcaaaggccctcaggcagggataagtttatgtgtctaaagaacagcagggaggcaagtgaacaaagggagagagtggtagatggggaaagagaagtacaaaagccgtgttgcccatggaaaggactttggagtttgtgtaagcacgataaaaagtcatcagaaggattttctcaagggagtgacatgttctgaattatatcttacaagactcactctgactgctaggagattctgggggccaaaggtggaagcagagagagaattaacaaagttaatgcagtaataaaggttagaactgacagtggcttggagcagggaggtaacagtcaaggagatgagaagtgattggattctagatatattttgaatttagaactggtcgttttgatggctgattatgtatgggataggagaaaaaaagaagtcaagcaactgatttcgggcaatctgctttacagatgaatggattattattgtctagcagtaaaagtaatgggggatgaggcatacagaaaacaatagaatgagtcagtgaaattcaccagactccccaaagaatcgttttggtcagtagttaaaacagagagctatagcagagagagagagagagaaaagaagaagaagaagaagatgaagatgaagaagaagaaaagagaaaagaagaagaagagagagagagagaaaaggaggaggaggaggagaggaagaaataacttctgggaggaagaaatcctacactagaagacctcaggctcttgttggtagtcattggagatggccttggaagcttctgaagctcatctactaaagaaaaatgtgtcttttgctgggaggcatcaaacatagaaatgtggatctctttcctcagggtagcctagcaaccaccagcctggcacagcacatcagcaatgcctatgtcacctattacggtgaccactccaaatccaatgccactggaatccaaaaaggaacttgatttttaaaccccttcctcttatttctctctcagaggaagtcagtcactacagcaagtatggacattgaacatccctttccagggaaattaccttgtctagtgatatggatgtctttacagtgcatcaggttggttaggaagcttttctccataacaatagagcaatgctggctgtagaaagttgaaagttgaagtctctttctactcaagtagtcaatgaatctactgtatatttctgtatattacaacattccagggctcctttgctggctgctaaccctcctcaccctgaactcagaagttacatcaaccattcatttacttacagtttcattgagatctaattcacataccatgcagttcaccactttaagtgtacaattcaatggatttttagtctattctgagtatgtaaatttttgttgatgtatagcatacatacagaaaacaggacaaaacataaatgaacagctgatgaattttcaaaatgaacatattcataaagccagctttcatcccgctacagcccccacaggcctcctcatgttcccttactggcattacacatccccaaggagagccagtatcctgacttctatcaccatagattaattttccctgttttaaaactttctaaaaatgaaatcttatagtatgtagtctttgtgtccagctgcttttctaaatttttgctgtgaaattcaatcatgctattaggagtatttgtaggatgatttattccccttgatgtatggtataccattaaggaactaaagttctttttttgtccatattgctactgatggatagctgtatggtgcacgattaaggaactgtaatttattttttgtccatattgctattgatggatatttaacattttcgtgtatgtgtttggagaacattttctggggcgtatacctagaagtgggtcatagtaatgtgtacatgcagctttagtaggtactgccagttttccaaaggggaatatactatattacactaccattagcaagatatgagagttctggtggcttctttacttcaccaacacttggtgttgtcatcaagctttctcaacctcatcttcctggactctggccagaaggcccctgagtaagcttcaagtaccttctcctggtgttatattatctatatgtatgcactctgctggagagacttcatggtttgcaacaaattttcagaggagcccttgtcccagagaagggcaaaaactacggcttccagttttcagctttcttataatctctaatattgtggtgaaacagccttttatttgagccaagatttctcctggaaaagctgacactggtagatagtcgtctctatttttgaaaagcacattattcaaggccagaacactctggagttttgctagtgctggtgtgcatgttgagcaatatgttggggatatccaaaaattacatgtcctaaataaagggatgatatttattgagatactttagatgcctgtgctatttgatcaaataaacacttatgtgtttacaaattgaaagagtgagaaagttggcacagcaaaaccaattttagtcgtgggcattattctgctttggaaacaacctcttggcatgatggcatgtcctgatggttagaaatgtgatacagttggaaatggctgatacagctgaaaatggctgatacaagcagcaaagaattagggtcataaaaccctgcatccttctgaacacacccttattctttgaggtcaatgcatggactaattttggagacttctgtggaactcaaacctgtctccactgacagatgcatttacaccagattatgagggtaaataggagaaagacaggtctttgagggaggaattacaattttcagcttcttaaacactttacttttttcagaataaattaattttgattgtgtttagaaagcagtcaaacttctgactcagactctgaagaattcttcttattttagtactgtttatccagtcatctatctatccattcattcatccatccatttccatccttacatctgtccatccaaacatccattcatccatccaaccatcccatgcatgtcaaacaccaattgaatatataacattcttaagcattatgggatgatacagatgattggttcatttcctgatatagctggagagggaagacatacccacatggaatacctagagaatacagtactatcaagataacatgggcaagtacaagttaagatggtagggactcaaatggagtgaactttatgtgcagagcactgatgggtagtgagatgaagcttggaaggcttcttgaaggagtcagtcttgagctttgcaaagaaagttgtttatactttgcgctgatggatattagaaaataaaaagcctttgaggaaagatgcagtgatgatacactggtgaggagaggatagcctgctgacatcagggaaactgcttgaccagagcacagaggcagccaccttcttcttggaaggcatcttcttcctggcagccaccttcttttggcagctttgagaaccaggcacaggagcttgaatttgttccagtgaacaaggggacagtccagttggaaaagagataagacaaggctgcccccttctggtttcttgtgcagtccattcatgctcccatctgaagacactagggcctctgcctgcctggagcattctcccctccagatattcacatgatttcccccctcacctctttcatctcttcattcaactgtcaccttctccttgaggccttccttgacatcactttaattaaaattgcaaccaacctcaaaccaccaacacttcctctttgccttccctgctactttgtcttcacagcacttttcaccttctaatctactacatgattttcttatctattttgtgtagtgtctgttttgtcagtttttccttgtttatacctactagaatataagctcccaggagagcagacttttatctgttgttcctccagtgcccagaacagtgccaggcagacaggaggcactcaagaaatatttgttgaatgaatgaatgaatgaatgaactgatgtgacagccattagaggatggactggactaggccttgcatgggaacaggagggacagccacaaaaatgatctggctggtcattgagtccgtcattagcttctaactagtttgtaagaatctcaagtggttacttgattaaatgccttccagagactatctttggaccacatgagaagtggctcatagagcagagacctgacaagagcttgaactctattactcatgtgcaatttattgtatgtcacttatgctgcaataaagctgtttaagaagaaagaacgtgagctctacctacacaaatctgaggttaaattcagtttctgcagtatgcaaactgtgtgaccttggacaagttactcaaccctatgtgctatgaaactcaactgcaagatgaaactatcagcagcttactcactggatctttgtgaggattaaatgaattaacttaaacctattagcccagtgtctgacaaatagtgttcaatcattataattaaaaggaaaggctgggaagcttcatgatcgagagcattggtctttgaatgtctgaatttaaatcctgctgccacatactagttgtgagatcttaggcaaaatataattatttatctctatatgcctcagtttcttcatctgaaaaggacaacatgatgcctatctcatagggtcactgtgaagattgagtcaatacatatgaagtgcacagaacagggcctgaagagagtaagcactcaatactacttgttgtcattattgcttcttattattattcttgcagggcttcacctggtttctcagccactatgactcccatcttccccatttctttctatgtggacaatcccaggcctttcacatgctgtggtgctgctggaagattccaaaaatgcagcattgccattgtctgcacctcactccagtttcacccatgtgatggtgcaatcagaagacagtgtcagtgccaattctgtgtgcttagaaatgttagcaagcaattctataagaaaaaaatctaataattatctgatcaaaaaatggacaaaacattttaatagacatttctcaaaagaagacgtccaaatggcaaatagacatatgaaaagctgctcaacctcattgcaaatccaaactacagtaagatagcatctcaccccagttaaaatggcttatattcaaaagacaggtagtagcaaattatggcaaggatgtagaaaaaagggaatatttgcacattgttggtgggaatgtaaagtagtacaaccactatggagaaccatttggaagttcctcaaaaaactaaaaatggagctaccatatgatccagcaatcccactgctgggtatacaccccaaagaaaggaaatcagcatatcaaagaggtatctgcactcccatgtttgttgcagctctgttcacaatagccaacatttggaagcaacctaagtgtccaccaacagattaatggataaacgaaatgcggtacatatacactatgaagtactatacagccataaaaagaatgagatcctgtcatttgcaataacatggatggaactggagatcattttgttaagtgaagtacaccaggcacagaaagacaaacatcacatgttctcacttatttgtgggatctaaaaatcaaaacaattgaactcatggacatagagagtagaggatgcttaccagaggctgggaaggatagtagaatgttggtgggaggaagataaggatggttaatggataaaaaaaaatagttaaagaatgaataagacctactgtttgatggcacaacagggtgactctagtcaataataatttaattgtacatttaaaaacaactaagagggtataattggattgtttgtgacacaaaggataaatgcttgagggaatggataccccattctccatgatgtgattattacacattgcatgcctgtatcatcaaaacatctcatgtaccccataagtatatacacctactatgtacccagaaaactttttaaaaatttaaaaaattggaaatgtgaacaagggtcatgaaataggcacacgaacagaagaagacaaccatttgcccaactacaatttgcaggacttctcccctcctccctgatgggaaagactaattttattttctctcaaactgcaagtataggtcaaaaggaaagcttggtccttcaaattagtttatggcccaagaacaacccttgttcataactgtaaaaatgattgagttatagaggggaaggtggcttaccctggctcccaacagttagaagggcaaggttcccatgaacatcagaggagacattctgagagaaaaaggtcactcctcaggaactgaatctgagaaggaccaggccacctgtttctactgacagggactgggtccagcatcaagaatatgatggcaaaagggcttcccaaatgtgacagaaattggggtgttgggtctttacctccagaacagaggtaagaaggggagaaggacatgtagaacattgatgttgataatagtaatggatgtgtgacccagccagcctgtttctgagagccactcactcactcactaggtgacaattctaggaagtggagttcaaatgttttaactgaacatacaggctccaaaatgaggccgtgtgagaatcagtttgcttactgtttttcagaaagtctgctttaaaaagtcaaagacaaattttcatggcaggaattcttatgctaggaattcatccagaggagattcatcaaaagtgtggtcatggatttatgggtaagaagtggttgtataaatgatggtacactcataatgatcacaaaaccatcagcaatatccatttagtgcatgcatcctgtgtaccttgtataatctccattattcctacagtacatccaagataggtatcatgattccaattttaatgataagagaactgaagcttacaaatgttgagcaatttgcctgtattcatacagctattactttgaagagctggttcaagtcagttctgttggtctcttaaaaatcatcgtgtaatccttctaatgagattctagtccagagcctctaacttttttacattcttttttttattattattatactttaagttttagggtcttaaaaattattaagaattccaagtagcttttgtttttgtggctctatctctctatacttgccatcttataaattgaaattgagaatcttaacaatatttattgacatgatttaattacttaaaataacaataataaccctactataagtaaacataataaatttttattaaaaactgttttctaaaacaaacaaaatgagtgagtgacattaatttacattttgcggatcttgttcacatctggcttgaagaagacagtgaccatggcagctactgtaaatcaaattgaacttccaatagctttcttttttttttttttttttttttttttgagacagagtctcgctctgtcgcccaggctggagtgcagtggcgcgatctcggctcactgcaagctccgcctcctgggttcacgccattctcctgcctcagcctcccgagtagctgggactacaggcgcccgccaccacgcccggctaattttttgtatttttagtagagacggggtttcaccgtgttagccaggatggtctcgatctcctgacctcgtgatccgcccgcctcggcctcccaaagtgctgggattacaggcgtgagccaccgcgcccggcccttccaatagctttcactcatgagctatgagatcccaatctagtcatttaaacttatctgagctatatttcctttacctgtaaaaggaagaaataacttctgctggacctacttaacagggctgctgtaatgatcaaagaaaaatgctatatgtaattagaccttttaacttaggtacatcctaggacaaggacttattctaatgtcttctcatgatttcttcagaagaacaagcctccctggacaatgttcaaaacagtaataatcactggaatgtttccatcatggccaaatgtgaggcacaaaactcttgcctcagattgtgtaatcttataaacttagacatttcctccttaccccacttactccctgaagcttgaagatttgcaaatttttatgagtctaacaatagctctttcctgtgtttatcagaagttttccctaatcttacaaaagaagatttgtttttatgaatttacctaaactaagctgttgcctgcttagacataagacaccaaggaggttaaagggtaaagtgttttattctgcttcatgatagtttcctttacatattgtttggttcccatttactcacacatttactctgtttttggttttagagtcttgagcaaacctcctttctaggagcattcctgagttaggagggctttaacagctggtctttgacaccattgcattgctgggattattgctatttgggcaaccctcaatatttttgggactccattgaatgagaatccgtataattcagctgaggtgacatttcaactgggttattcagatgggatctgtcaaatagagtcttggaaggggccccttcccaccctcatcacagcatttccatatgacatgtactgtacaaataatttatctctggggaaaggaaggagggatggtggagaggtgcccatcttatgtgttctggtgggaggttaatatagaaggatatggctgggtgcggtgactcacacctgtaattccagcactttgggaggattacttgaggtcgggagttcaagaccagcttggccaacatggtgaaaccacgtctctactaaaaatacaaaaattagccaggcgtggtggtgtgcacctgtaatcccagctactcaggaggctgaggcaggagaatcgcttgaaccaaggaggcagacgttgcagtgagccaagattgtgcaactgcactccagcctgggcagcagagcaagactctgtgtgtgtgtgtgtgtgtgtgtgtgtgtctatgtgtagatatagatatagatatagatatagatatagatatagatatagatatagatatagatgtgcaggatgcttttgttgggcagggctccacatgcaggtcatggttagttagttaactctgccttgttccaaaagctgtccttcactttttcccaggccaagtcccatgtgtcagactgagctctcactttctgaatcaattgtctttatgtttccaggagctgccatggttgctggtgcaggccctggcagtgacagacagacattaattaaccacatctgctgggctcacattcttcttcaagtcatctggtggtgatttctggctgaaccaatgcatttgtgaaaacaagcaaacaaaaaaacctaaataatttaattgtttggctgaatactgatttcttcctatctttttattaatggattttcaagcaaaaatatgctgttcttcccacttatggtgtggctatttagctgcttatggttttatctctttgtgattccctttactcgtgggcacaatgccacactgatagtgcagaaggatgactttgtacaccagtcatagatgcacattgctctcaatgtgcatcttgatttggttctttgctatttaagttccatcccacacccactttgtacaagtgcattgtgttgagggggcagggttgggcactactctgctggtagggatctgcagagaccatagtgggtctgggttcaaggggagacttaaaacaagtaggatagatagttataacataaggaaccaaagtacaaaagatcagtttataaatcggggcattgtgtgtcaaataaatgacaagttcaaggtcacacagctgagattatatcaagcatatattgtgaacctactgtgtgccagcagtctctgccagcacgtcctaggcatacaaagattataattataatagtagcagctgcggtaataatattgattgagaacttacaacatgccagccactgttcaaagtgatttacatgtatcaacacacttcatctttctaacatgcctccaagacagttactatgatcacatttcactactgagttaactgaagcacagagaagttaagcaacttaacacagctagtgagtggcagaccatgactcaacccagggagactggctccagagcccatgctcttgcagcgtagggcccagtgaatgagatagaatagtaaatgcatgaaactggtgcagtggagttagcggcagatgaaagagaaacagagagctctgggacactgagaagaccacctaacccaactgtttatgctaatctgggcatacttcctggaagaagacgatggagtcaatagatgttgaattacaaagactgatatctggggcctggacgattaagtaactgtcttactctgtgtcagtcatcttaggagaggcagagctagaatggggattgacttcttcttcgtggagaatggtccctggatcaatccacaggtttctgctgagcaagttttatgtattgaactctgatgaaggagggataagtggaggttttcaggtcagcatgcaagttgtatggaacatgaattatttctcaataaagctgattataaaacaaaatcagcatgcactcagcagccagaacttgcttctaaataccactctcttgataaaaggaaagccttcttggacaaatgacagatcctagggcttgggcagagaaaatagaagatgagtctggagaatcttctagtgccaaaaatgaaaaaaatgctcaacagacaaaaggatggggacatgtcaaagggactcaggagccgacctgaaggagtgctcagaagtagaataatttgagcaacaaataaatcatattgtattagattataacacaaggtataaaacacatatatatgtccactgttataaataaatgaatgaataagcaagtaaaaggggaaaagaggaaaatcttccttagaaaagaattcaaaaaatttgtggggattctccatctccagaaagtggaagttagctcccaccatcccctcttgaggatgatctgaacttaatgactctcttccaaagaacagagcatggaagaggggtgagtagcaactctacagtggagagacctgacagacaccaccctaagcaaggaatcaaggttaacatcatccgtgataagtcatattgatatcaagtgccctctgaggtgacatgatgacaagagcacttggtctttgtggtagtcttccccaaaattcatagtcctaatctaaaaatgaaaaaagtaacttcagacagatccaaattaagggatattctaccagataactgacccgtattcttcaaactttgaaggttatgaaaaataagggactactgagaaactatcacacaccataggagactaagaagacaggacaactaaatgaaatgtggtatcctggatgggatcctgcaacagaaaaaggatggttagtggataaatgggtgaaatccaaataaaatctgaagtttagtacatagtgatctaccagtgtcgatatcctggtcttggcaatgtaccatgtaatgtaagatgctaacattagagaaaactaggtgaaaggtatatgggaactttctgtactatctttgcaacttttttataaaacaaatattactttgtaaaacaaagttactttgtaaaaatttgtaaaacaaattactttgtaaaaatgtgtaaaacaaatagaaactatatttaaagcataaagcataaaagaaaagtcagcaagtgtcagtattctgatcaactagaactttcatgcattgctgttggtaatgtaaagcagtgcaacaactttggaacactattaaacttaaaaagttaaacatacacccactgtgtgactcagccattccactactaggcattgacccaagagaagaaaaaaacatatgtacacaaaaagacctgtacaagaatgtttatagcagttttgttcacagcagatcaaaactagaaatagttatcaacaggtgaaacaaaccgtgatgcatccatacaatggacactacttagcaataaaaaggaacaaacggaaacttggacaaacctcagaaatgtcatgctgagcaaaagacgccagatacaaaggtgtacatcttgtatgagtccattaaaaaatgtgaaaacaggcaaaaacaatctataagtgacagaaaactgaacagtggttgcccagggccagaaaggggacagggattgtctaggaaggggaaagagggaactttctggaatgatgggaatgttttatatcttgattggagtggtagttacataggtgtacacatgtgtcataactccccaaattgcatgttaaattatttaatgtgggtacatttgtgaggagatattggtcaaaggatacaaaatttagttagataggagaaataagttcaagggatgtattgtacaacatggtaactatagttaaaaacaatgtattgtagtcttgaaaattgctaagagaatagattttatgtgttctcacctcccaaaatgataggtatgtaaggtaatgcgtatgttaattagctcaatttagccattccacagggtatacatatttcaaaatattatgttgtgtattgtaaatatatacagttttaatggcaggttaaaatttttaaaattacttctaactataaaaaacaaaatacggaaactaaactaaaataaaatgagtacattgtagctaaagtacacctcaatagtgttaagaagggtgacagttaattttatacgtcaacttgtgtagatatttggacaaacattattctaatgtttctgtcaagctatttttaagataaggttaacatttaaatcagtagactttgagcaaagcagattaacttccataatgtgaatggactttatccaatcagttgaagtccttaagagaaaaagattgatgactctcaggaaaagagggaattctgccagcagactgcctttgaagtcaaactgcaactcttccttgggtccgtgacctaccctacagattttggacctgccgtccctctcaatcaacatgagctaattccttaaaataaatctgaatccttctctctttctctgtttctctctctgtctctgtctctctctccatctatatctatatcaatatcatctatctatatctatgtatctatgtatctatatatctatgtatgtatctctctctctctctctctctctttctcctgttggttctgtttctctaaggaatcctggctgagaagaaacataaagctgtatctcaacccttccctgagaatcttatggccttgttggagagagaagaccaacatggccacagaattaatacaagaacaaatacgaaatctcttattccacaattctagtttctctgcctgtacaacatcaacagaaggtgcatctttattgaatgactcagagttttggggaagtttctgttgactgagaaccttaagttattctgattccgttgaaagatgctatcagaatgcacgacctggcttctgactcgggttttcagattgacccaaagtgggtttttttgcgtgtctcttaagtgccatcaacaggttaattctcccagatattatttattttaaatccttggaacaatgtgttccctttatttctgtgtcgaggtatccctgtgggaagaaccaggtggtataacatgtctagaagagaagtttgaagttgtctaatctttctgctttgactttgctgatctctgggaactcctgtgtttacctagcacatctgagtccttgggaaagctttctgggccctgttttgtggttcttctaacagatggttgcattcttgtgattgatttttgatccccttctaagttgtataatgcttatagttataattttctgactctccaggcacacagaggctcctgactctgagatatttgcaagtaccattgacaaataagatttccttaggttaactccacttatgtacttgtatttacattttgtatggtaaaggctccagtttcagagagaaacctctttaccgtgcttggtgtggcagtgaacttaattaacagagaattttgctggcaatctctatgctaaaaagttaagtggggttctgaggacacaaggagctaaaaagttgagtgtatatcacatattgataactcacataattttgcttgcagacatttaccaatttggcagattacctacttttacattgtagtaaatatttccttttaaaaatatcttgtatctcacagggcaaatcataccccttcagggggccattcccacctgtatggaatccaattacctacttagatcataacaacttttggaggacaatggatgacatggggcgagaggtaaagcttctttgactatatttgtattcttttttgtaataagtttcatccttcaaagaaagaaagtaaaatatatctccaacacctagcacattgtgaacacatggtaactaaagatttgtgaaatgaatgaatgaacttgtttctaacctctgcaataataagatgtcaaacagattgatatttgtatactactgatgagtgggcaggagattgggtgtcactcagccttcttggaatgatgtttcaaattttggaaatcttcagtacatagcaaaattagacttctgggtctttgattcaccaccatgcccaaacaagtcataagtaatcacacataaagcattttttttcttttactttaagctccgggatacatgtgcagaacgtgcaggttcattacataggtatacatgtgccatggtggttttctgcatctatcaacccatcgtctaggttttaagccccacatgcattaggtatttgtcctaatgctctccctccccttgccccccaacccccgacaggccctagtgtgtgatgttcccctccctgtgtccatatgttttcattgttcaactcccacttatgagtgagaacatgtggtgtttggttttctgtttctgaacacacataaagcttaactgaaaactccatagacatgatttgctgcagctctgtgatccttgttaaatagttaaatttatgagtgttctctagaagttagtaacttaggaatccatatctagaaatagcccagttacaacatgcctctatttattgtgcaggaagttttatcacaaattaaatatggcttgggtggtacagatttataataggaaagctacatagacagcattgattatgcagtaaaagcaatattggatgaatttggaaaacttaacatttttcctctttaaggtagagtttttaatactatttgaatagttatttaaagtggaaaattacaaaaatgaataaaataaaagagaaaattacatttgtctttctccttcgaatcctcatctgaatgtagattccgagtgatgccccatggaaggctccccttgcagaagagtgggacaacatgacaatgaaggagctactggacaagctctgctggactgagtaagtcttgccattaggcacaggcatttactgtgaccaccttttaggtttatttagcaataccgttcaacaagtatgggacaagtagctgctttgtgtctaaaaccacaccaccagccagtggcatgctgaaaaccattggaattggctcctaccctgaagatatctgtacatacaacttacttctttggagtagttttgtatcacaaaggtggtattaccctgtgaagtcctcagaacagaccagaaggtaccactttctttatctgaaacagcttaaagaccatcagcttaaagctctcatttattaagttgttgatataggacaatttttgtattcttcactggtggtcaaatgtggagatggttagcatgtgcatttgccacaccttgtgtgaagtagtgcaattcttcaaggacttaaagaggaacctctaaagcctttgtgtagataggtcacaactacaggggaaacatgtgtgactggactggctgttcccctttagtgaaaaaacaagtacctatgagttaagcattaaattcttgttggcagaactgggaactgtagagaaattgtgaaggcttgtatagacagaccacatggagaggccacactgctcttggacagcagggaaaatggaaaggattatgagggttcccattcaagcacgtggtaaatttgtggtaaacaaaataagagaaatggaagccaaattcaaggagactgccctgtcttgctaaagagcattagttgagaatatgtttggctcgggggttaatgtcttcatttttaggcattcattcactgccaactaaaagtaaaaacaagcttttagaatatctgaatcttaaaaatggaaataatcaaaagacataaaattcatatatttttcatataaaaattcagcttctaataatttagctttaagaaagtgaggcaaaagaagagagaggcaccagcatggcacatgtatacatatgtaactaacctgcacaatgtgcacatgtaccctaaaacttaaagtataataataaaaaaaaaaaagaagagagaggcatacagggagagaaggagagagggagagggagaaacagtgaaagaggcagattcaaagcattatttttaaaagggaggatctgaaagcccaatagtagaagatcggcagaatcaagtatggaacatctaaaaaattgagtacttgagggttttaaaaaatcgtgttgtagaggaatatttaatgactggaaaaaatagtaatattaaacacatagaaaagcaggctattgtggtatggtatatgatctcatttctaaaaacaactatttatatatgcactgcaaaagcaatggacatccattgaagtatttttaacgtttaatattaccatgcaaacatttatttttaaaatgtttaaaaactttacatcattaaaaattattctttaaacatcatatttcatggtaccagaatattccatgggaaatgaatacgtaatgtatttgtccattatcatcctgttgaacacattggttactttctgttttttgttattatcattatacaatactctataataaacatctttatgcctctcctgtgttttcaacctttgaaagcaaccagttctggaatagtaaaatccttttatgtcatgaaatcaatgcgtgttattaattatattcttttaaacatttacctaatgctatctaacacctctatgagaatgtagtttgcaatataatttattttaatagtaataaaattgtagtatttagttttaaattatatactttagattttcaaaatataataagtatgtaattatctgcatttgttttataactcctgttatgaaaagcttttaataaattcagttaggtcttctctcctcagagaacttttaagtttcttggtgataaaatcaatcatatgtttttgggatcacagggacccgacattttctatcgtagcccttggcctagtcctccacttagtgaatattctaagttgtcatttgacaaaataaagcattctgagatactaggagtataagaacacaagacaattttccaactcttcccaagcaagatacacacagtattatttcctggatttaaatgaagtaatccccagaatatccaacctattgttgttcaaactaaagcacaatcatacattccaagactaatgttgattattctttcagttattatcatttacaaagtgcacttcacaaacatgaattgtattttcaatgtgatcacagctatgtaaaaacattttttaaaagacctatacttagaaaaaaatgcatcaaaatgagactagtaattatcttctggaggggcagaaatatggaagacactcgttctctcatccttttatcttataaattttccaaattttatataatgtgtatgtatttttcatgtagaaaaatattataacatttatcttttaaaaagtcaacagggcaaaaaatacggaaatattgcactaacttccttgaccttccatccttcaaatattgttcttatttcttttcttactgaagctcctagagtaaattcaaataaaggattaggaatggactggcccttcagaattacttttagatctccctttatttcaaaccagaattatttctttcccaccaaattgccaacaataacaactagaattccagcaatatttttgttaaatattggctctccagctgggccaatgttaggtttcagttatttattactccctttactgtatgcccctcaatccacctaaaaaataaggaagaaaagaaataggattttaggaagcaacaaataaaatactacttttattttaaattgacgtctggatatgtgttttagttagatattacaaattgcctctgcaaggaaggcatgagctagcaatttccatcccttcaattatcctgagaaatcttacaaaactaactgtaagtcgctttaatgtatatatgacaccatttcacaggctgtaatgatggggactgtcatagacgggctgtcaggttgttacagctgcaaataatgtcaataattggtatgtgtgttaggcatgattctacaaacttctagggtcaagatacagtaaagtagagagatgccccttggtgagtagctgcacttccaaggctgtcagctgactaattagaaaacattttgaggtatcaaaagcacgagttttgcgtcaagtacgatctgacttgaagttgtgtcgttatatattcctaaactgtccgagactccgttttctagcatgtgaactgtggaaaaataatagatatttgatacggttgttgcaacaatttaacaagataatgattttaaagacaatggagtgtggaaagagttcaataaatggaagacaatatcatttatcccaaccattgtcagcattaccaggtggaaaatgctgcctcagatataacaagattaacaatatgcaaacttcatgtcaaagtcaaaaggggaattggaccttattaaagaaatcccagagtgcacactactactgatgaattttatgctgtgctagatataatggagtcctcgaaattgcatgagatagtttgctttctggtgtgcttcctgataggtgataacctctcaccatttacctgccaatgtcaagcaaaagcttacccatttatgctctattaattgtttgtcccctcatccattatttgagcttgtcttctgttaggcagtaaaataactgaatagataactgtgactaattttgtgtttggtacagcacctagcatatcctttgcatgttatggatgtttaaaaaattttgtttaactgatatttctcatcaatcattcattcgttcaatcatgcaacaagtaattattgagtgcttacaatgttccaagcactattttgttaaaggggacactatggtgagtgagaaacagaagatccttgttctcataggttgatattctagtggggggagacagcaattaaaaagaattaaccaataatcaagacaatttcagacagtgaaaagagttataaagatactatacagtagcaaaatgatagagaatgtcaggatgctgggaatatggaagccagtggtcgttttcatagacaaatgtgaatatgtctttctaaggaaacattagagtaaaaagaagagggtacaagatgagacagaaaaggtaggcatgggctggatcacatagggctctggaagccatggtgtaagatctgaatcttattctggttttaataggataccactggagactttttaagcaagaaaatgacatgatttgatttatacttcagagagagcatcatggtagggagggagggaaaagcctctggctttgagtgtggtgaacagataccaggtgaggatgaatggaggcagagaggccagtctgaaggaagtaattgcagtactcctggaaagagatggattctaaatttgtggtgaaggtggagtgatgtggtgagagataatgggacttcccaatgaattggatgggggaagattgatggaaagagagaaataatgtttgatttctagagtgttggtttttaccactgagtaaatgatggtgctttttactgagatggggatcactggaagagcagcaggaatgtaaggagaaatcatgaaagcacagaatctggaatagaagctgattctgagtaaggtgttttgtttacagggaaaataatctgatatttcaaaaacctccgatgtcacgttttgtaatattagattctagtgacaattttttgaccttaccacattgttttaaacttaaccaagaaaatgtgttacttaaataatttttagagaattaagaagctgctctcctgcgtttgccaagtttgctcttgtttcttcctgtgcagatctgcaaagcagcttgccactctctttgtgaacctgtgtgtcactgcagagacccatgaggtctctgctctctggttcctgtggtatgtgaagcagtgtggaggcacaacaagaatcatctcgacaacaaatggaggacaggtacccatccattcttccacagtcccaatggaaaaacactgctactgaaatgaaagatcatcatccttcaatcatgaactgctgaagtgggaagcaggcttgtggcttttagagcattaccatggcagctcaaagtgtttcttgtaaggcagtctgttgtcaggtacccactgtgagaacccagtgtccaatgtaattttaaagctaggcttgtctctctttatgcactgtggccattttccatacgctcaattattatttggtaagtttgtaggagaccatctgaattaagcttagcttgagcacttcttggaaagcttataaaggaaattcagtaatgcattttcaatttaaaacacacactattcatggaattcatttatctattcattcattcaatgcccatttcttgagccccggcactgtataaggcactgtgctagacacagtaggaacatattggagttcttaaataatctgcttggttgtcatgttccattcttctctctccccctcctcctcttctttctttctcttctcctcctccccctcctctttctcctcctccttttctctttctccctctccttctccttctctgaccttaactgaaaattgaggaggaggcagccaggtcaactgtgtgcatagccaggtagaacatttggaagttttagcaaggctgagggcaggtgggtacagtgaggtgaaatgagttcggtggctacagaagcagcaggcatctgacccaggataagatgggcagcctgcaacagggagtaggctggcctgggggaaggggacatggtgggaggcagggaagttctgcgcttgagccacaaagcaaggggaagcaggcttaggtctgctcaggcaagctagggaagagctttaggtacagcttcaccagttccagctctaagcaaaagactgcagataggacagagagcagggatggtgaccagaaaggtgggatacaggggtcattctgaagatgtccagctaaggttggagtctgggaatctacaagagcatagcttgtaaagtaacttagaaatcctgtaactttgtccaaagacagcaattcctacttagaaaaccatggtgaaagccactattcactgcagcaaaatgaaatgttagacatctcagagtagacatatgtgaggacaactaagaatttagcaatttatgcccattcctgcgtttctctttcacctccttttctctttccaggagaggaaatttgtgggcggatctggtcaagtgagtgagcggataatggacctccttggagaccgagtgaagctggagaggcctgtgatctacattgaccagacaagagaaaatgtccttgtggagaccctaaaccatgagatgtatgaggtaactgtgatattgtgaaatatatatttgatcttcatcccagtttcctggcatacaactttaaaaattcttagaatctccagagtgatgtcctttgatgccaatgattgatggctggcagcccctaggtagcttcaggatggggctggtcacaggaaagaccatggaaagactagagggttgggactttcagccccacccccagcctccagggaggggatggggcaaggggctgaaggttgaattgatcaccagaggccaatgatttaatcaattgtgcctacataaggaagcctccataaaaacccaaaacgaccgagttctgggagcttctggatatctgcacaactggaggttccttgagaatggcatgcctggggagggcatgaaagctccatgccctttctcacaactcttgcccaatgcacctcttcctctgtaccctttgtaatatcctttataataaaacagtaaacatgtttccctgagttctgtgagccactgtagcaaatcaatcaaacttgaaggggttgtaggaacatcaactggaagcagattggtcagaaattctggaagctggacttgtgactgacatctgaaggtgggggacagtcttggagactgagccctcaacctgtaggatcagaagttatctccaggtagatactgtcagaattgagttgaattcagaggacacatggctgatgtctgctatagaattgcttgcttgcttaatatgtggggaaaaaccactccacatttggtcacagaagtcttctgtggtgatcgttgttgagtgagagaatggaaaaaagcacttttttccattctctcactcaacatttgctttgaactcaactttgctttgaaatttttccactcagagttaccaagacacttaaacaagtgggaagaggccacagtctcatagataatcaaagccgaagtcaacaatgtcacacactttatagacagtctttttgccaatagtgaaaaagctatctctaactgaaaaaaaggaaaagagaaccagaatatttggggtgggggaggatttataaaaacttataaaggtattatcaaccctctgtattttgcttttatgtaattagaaaaacacagaaaatatttatttgataaatatcaagcacctcctatgtgcctgacatgattctaggagttaagaacacagtcgtgaacaaaacagatacaattctctgcccacatacaattctccttctagtgaaggagaaagacagtaatgaaacatatagttataatataaagtatgtcagatagtgataattagtgcggaaaaaatcaagcaggaaggtggggagagggcataccagaaagtgagatgggagaattggttatgcaagtttaaataaggtgatcagggaaggcctcactgagaaggtgatatctgatagagaattggaggagacgagggattgagccatgtggttccctgagagaagaagatggaacagccagtgccaaggcactgaggtgggagcaagcctggtgtgaccaaggaacagcaaggtgatcaaaatggcagggccaggcttggtggctaacgcctgtaatcccagcactttgggaggccaaggtgggcagatcacaaggtcgaaagatcgagacaaccctggccaacatggtgaaaccctgtctttactaaaaatacaaaaattagctgggtgtggtggtgcacacctgtagtcccagctactctggaggctgaggcaggagaatcgcttgaacctgggcacgtggaggttgcagtgagccaagatcgcaccactgcactccagcctggcgacagagtgagactgggtctcaaaaagaaaacaaaaatagcagaagtaagagtgtcagggcaaatgtaacaggaggtgagatcagtgatgtaacgggcccatttcatgtgtggccttggcgatgatggtgagaaatctggctttgactttaagtgcaatgggaagtcattggaggttttgaactaaggaacaataagggctactttaggtttcgacaaaatccttgtcacttctttaagagactgaaaagaatataacgatagaatgagagagaatcattgggaaaaaaacaaaagcaacacggcaacaatgtttaaccatgttgcttttctttcaggctaaatatgtgattagtgctattcctcctactctgggcatgaagattcacttcaatccccctctgccaatgatgagaaaccagatgatcactcgtgtgcctttgggttcagtcatcaagtgtatagtttattataaagagcctttctggaggaaaaagggtgagtactttccttatataaaaacctttagaagaaggtccaagaaacttgttgctaaggcatgcattttttaaaaatgtcaacttttattttagattcaggggtacatgtgcagatttgttacatggatatgttgcatgatgctgaggtttgtggtatgaatgattctgtcacccaggtagtgaacatagtaccaataggtaggttttcaactcttgctgtactccttacctccccctttagtagtcctcagtgtctattattttcatctttatatccatatgtaccccatgcttagctctcacttataagtgggaacatgtggtatttggttttctgtttctacattgattcacttaggataatagtctccagctgcatccatgttgctgcaaagaacatgatttaattctctttttatggctgcatagtattccatgctatatacataccacattttctttatctaatccacctttgatgggcacctacgttgattccatatgtttgctattgtgagtagtgctgcgatgaacatgtgagtgcatgtgcctttttggtagaacaatttatattcctttgggtatatacctaataatgagattgctgggtcgcatgatagttccatttttacttctttgagaaaactccaaatttcttttcacagtggcttaactaatttacattcccaccaacagtgcataagtgctcctttttctccaacatctcttattttttgactttttaataatagccattctgactggtgtgagatggtatctcatcgtggttttgattggcatttatctgatgattagtaatgcagagctctttttcgtatgctttttggccacttgtatgtcttcttttgagaagtgtctgttcatgcattttgcctactttttaatggggttatttggtttttgcttgttgaattaagttccttgtagattctggatattagacctttgtcagaggcatagtttgcaaatattttctcccattttgtaggctgtgtgtttactttcttgatagtttcttttgctgtgtagaagctctttagtttaattaggtcctacctggcaatttttgtttttgtttcaattgcttttgaaaacttaaagacatgtgtttgcatgtaactgttttgttagtatgctggacataaaatgttaatccaggttctaagcacagttctttcaaataaaatatattggcacaaactcatggaattaactttctttagaatataaccaactctttgtaaatcaataaaaggtttatttaatcctcccccaaaatcttgtgaaaagagatgagtaatcttttctaattcagtgttttaaagtatgggtttataaagccaatcaccaaggttgagattctgaaaatgtcttggctctctctcactagtgtcgattctaccatattaaattaaattcatttattcacttgcacatattcaacaagtgtactactcaattgggcagaacattgcagggttgctcactaaagtgctggattctacaatgatgggaatgttctagagctgctttaatacactagtcactagccacatgtgggtactgaacacttgaaatatagctaatgagacttgggaatcagattttaaaattctatttaattaatttttttttttttgagacggagtctcgctctgtcgcccaggctggagtgcagtggtgcgatcttggctcactgcaacccctgccttccgggtttaagcgattcacctgcctcagtctcccaagtagctgggattacaggtgcgtgccaccttgcctggctaattttttgcatttttagtagagatggggtttcaccgtgttagccaggatggtctcgatctcctgacctcatgatccacctgcctcggcctcccaaagtgctgggattacaggcataagaattctatttaattttaattgctttaaatataaatgcaagtagccacatgcagacagcacaacgctagaatcttgtcatatttgctcttatagaacccacttttcttccaagtggaggccatgtaagaagagtcagtatctagaacggagggtgaagggcgggatgtactccaaggaggagcaagactgcagaaagaaggttggaggcaaatggggaaagtgccacaattttggcttagggtgcttcttcctgtgtaactactctttttccgctgcatcacaggctcctcattctccacattgcagataatcacgtttaggactgctattggattggtgcatcagttgggcaagtaatctactgtttgcaaagtcagtgcagtgacccaccacaaagagccctgtcattttagtctttgaatctaatggctgtaacacactggtgctgaatctcttcctcttgtgacccaggccacccattttaaatgactggctggtggcaagtagataaggtttaggaccaggaatacagtcttctctgaatgagcatgggtgcctttatttatggagagaaactgtaactttccattcatgcctgcaaatctttatcttaggcctgctatgtgccaggcaagttgttaggcactagtatcagaaagaaaacccaagacctccacccctcagaatctgacttggtccttgttggtaatgagccttgcataagacttttaaaaaatgattgtgggcaaggcatagtggtgcacacctgtggtaccagcttctcgggaggctgagactggaggattgcttgagcccaggaggtggaggatacagtgaatgagctataattgaacttcagcctgggcaacagagtgagactccatctctatctcaaaaaaaaaaaagtttgttgacatgagatagcctcaccaaagcatttgagatttcttttgagttacaactttaatgtatttcttcaactgggcgcctattgtatgccagacacagtgctaggcactgagaattcaaaggcacttttccttgcccagaaaatccaggctcaggaggaagacagtcatgcaaactggtaattgcacaatgtattgagttctaggctattatagaaacaccaagtagggctccagactcacatccaatatgattcctgttacattgataagtgtattcaatgacacttatttgaaagtttctgtaatgaaatctgaagaagttcactcttataacaagatctttgctttgcactagactatcaacatcactgccaaagacactgtaattaactagtaacatacaagctcagtcaatatgaggtaacaagatagaagggtatgaattaagcagccccaacaatccagcacagtgattagcacatatcaggcacacagtcagtaatcaccagagttttggttttatgttgctttgttttgtttcacaagttcagtgtggcttgggttattaaagagaaggtaacattttgtattttgatacagacagtggtagccaactcttgattgcttctcccctccacaccccccacccaatcccagcatcatgctaaacactgcttttattttatttttaattgtagatatttaaggtgtacctcataatgttttgatacacatgtacatagtgaaatgatcttgtggtcaagcaaattaacatacccatttcctcacatggtcatctcctgtgtgtggtaagagcacctgattgcttctagattgattatcccaggaaatgcttcccagtctcttagtgtgtaacatctttgtgaatttgcaaggacaggcttcctatattttgctggccttccactgaggcattctaagtctagccgccctcaccgtcagcaccccatcctacacgggatgcatcagcccttcattctagcccacttctgtggaaaggataggctgttagcaatgcattgaattcttgtggtctccttgcttttgttcatctatgaaccatttctactttcccttgaatatttacatctaatttatctcaatttatgttttcaatggcagaagctgtacttgtttttctaaattacagaaataaatataatgaccataaaactttcaaaaactgaaagtatgtgaaaaatgtttctcttctattgttcctccccctagagggccactgttaaaaatttagattgtttatccttaaagatttactgtatgcataggtaatacaagttgaacatccctaatctgaaaactcaaaattcaaaatgctccaaattctgaaacttttgaagcatcgacatgatgtctgaagtagaaaattccatatctgacctcatgtgatgggtcacagtcaaaactttgtttcatgtacaaaattattaaaatatgtataaaattaccttcagactatgtgtataagatgtatttgaaacataaatgaatctggtatttgggcttgggtctcacactcaaatctcattatgtatatgcaagaattccaaaatctgaaaagagccaaaatttgaaacacttcttgtctcaaacatttcatataagggataaggatactcaacctgtactttaaatatatgtgtgtgagcatccctatatatatgtagagagaactatatatactggaaatacatgttaaataatataataaatattttatacaaatataactttaattttaaataaatatgttaatatatttttccaaaaacatgttttttaaaaaacatacatcatacatatcacactgaaatttgctttttcctgttaacaatatgccatggacatctctccatagcagtacatttaaatctaacccctttcgacaactgaataaacagtatctcattgtgtgccttatcagaatttacccaagacatcagctgttgatagtcatttttcttgtttccatgtttttgctattatacaccatgctgcaataaacagcatcctccatatagctctacatatttgtataggagcatttctttttgataaatgctgtaggatggaattatcaagtcaattgatttgggtagacctgtgaaatttttgttagggtctgtcctctcacatccttgtcagttgatataagttccatatctgtcttctccaaatctcatgttgaaatttgatccccagtgttggaggtggggcctaaaagcaaatgtttgggtcatgtggacagatccctcctgaacatcttggtgccgtcctcctccctgaggtaataaatgagttcttgctctgtcagttcccatgagagctggttgttaaaaagagcctggcacttccctcccctctctcttgcctcccgtctcaccaagtgatctgcacacgccagctcctcttcaccttcagccatgagtggaagcttcctgaggccctcatgagaagcagatgctggcaccatgtttcttgtacagcctgtagaaccatgagccaagtaaatatcttctttccttcatatattacccagcctcaggtatccctttatagcaacaccagcagtctaagacaccagctaataatatttaaaatttttttgtcaatcaggtaggagaaattgcctcatttatctataatttgtaatttttatcattaacaaagtatcattttgtaaattacctttgctcattaaagtttttttctgtttatattgcaaatattttctcccagtgaatcagtttttaacgatttgttgtatgatggtttccccctactaaattctcagatacacattgattctttctgttccactgacctttttcactgcgttctaaacatttttgcagctctacttattaaaaaatgtacacataaactatcactataggtattcctaaattgtacacaagtacctctgaaaaattatatcgttgtaactataaaacatttgaaaagtagactttttaaaaagcttaaattgaaaaaccagaatctctagtattttcttccactatctagatgtgcaatctaggtgtacacccccactttggaaagcacaagtttatattatctaatcctatggcagcattgtactgttttaatatctgtagctttatgatatgtttataatatgttatatattatgtcaggtaggacattcccttattattatttttcctttaattttgtccttggtaaacttcttcagttattcatccagatgaatgttattatcatctcatcaaagctcctgcctccacacccctacattacaaaagcttctattgacttattttattctgaacatgcctctttgttacctcccagagctacaatggcttcttttctctctgagaaagttagcactttgggggaaatttcttctactacctgaattattgggtccctccccctacccacccccccatagtttttctgtttcatttgttagttgtgaatttgtttcttctttgtctttgcatttattctttaagaacttctttaagtgtttggatgtccttgaatatcatctctttttctaagagtaaagccctacaaagctgatgagatgttttgtgtgcatgggtggggctcttgagctttctatctgcaagtggcagaaatctcttccatgctgcatagcttgtcctggcatgaacatgacttttctctctgctccttgttccttcacctccattaagtgcactcacttgactcagaggccagattcactctgagaaggaagtgtccaaggagcccctacatcgagaaagcagtacttccaccttggccagcctggcatcctatgctggtcctgtccaaccgatccccacatgatcagtatgcacacgttctttgatcagatcttgtcctatttgtctgctctctctcttgccttcttatattaggggattcctaagatggttctcttgtatttttaaaccttgagctcttagactttaaacatttcttcttcacatacttcagactttctcaacatcttttcctgccccagcatgcctgaaggacattcaaacacccctcaagccagtggcagattgggacattgattctaacaggtgcacagtggggaggggtgcaggagacgagaaagagacaagttccctttaaaaggcttcctggtttgtctgcttacacacacgtatgcacacatgttggggaggtcctttctctgttctttcttccttattttgaaatcttcttgttgggttttctatacaacatttgccgctgagtcttccacaataattttgttcaaacaacctcaattttgcaagtaaatgatggagcagaaggagttggacactgcagtaatatattgttataacatttcagactctgccctgatattttcaccagtgccctgtcacagtcttttgaaattgcatatacaggcacacctctttttattgaacttcactttattgcactttacagataattgcactttttacaaattgaaggtttgtggcaaccctgcactgagcaggtttatcggcatcatttttccaacagcgtgtactcactttatgtctctgtgtcatattttggtaattctaacaatatttcaaactttcattattattatgtttgtcatggtgatctgtgatcagtggcccttgatgttactattgtaattgtttaggagttccataaacagcacccatataagatggcaaacttaatcgataaatgctgtatgtattctgactgctcagtcaaccaactgttcccccagatctccccatcttcttgggtatctctgttccctgggacacaacagtaatgaaataaggccaatgaatgaccctacagtggtctccccagtgttcaagtgaaagaaagtgctgcacatctcttgctttaaatcaaaaactagaaatgattaagcttagtgaggaaggcatattgaaagctgagataggctgaaagctaggcctcttgtgccaaatacccaagttgtaaatgcaaaataaaaattcttgaaggaaattaaaagtgcactccagtgaacatatgaatgataagaaagtgaaacagccttattgctgatacagagaactgaatgatctgaatagaagatcaaaccagccacaatattcctttaagccaaagcctagatccagagcaaggcccccaactctcttcaattgaagttgaagctgcagaagaaaagtgtgaagctagcagaggttggttcatgaagtttaaggaaagaagcctcctccccataacataaaagtgcaaggtgaagcagcaagggctgatgaagaagctgcagcaagttatccagaagttctacgtaagaacattgacaaaggtggctacattaaacaacagattgtcttgttttgttttgttttgagatggagtctcactctttcacccaggctggagcgcagtggcgcgatctcggctcacggcaacttccggctccctggttcaagtgattctcctgcctcagcctcccgtgtagctggggttacagtcacacaccaccatgcccatctaatatttgtatttttagtagagacggggtttcaccatgttggccaggctggtcttgaactcctgacctcaagtgatccgcccatcttggcctcccaaagggctaggattacaggcaagagccaccacacccgaccggaaacaacaggtttttaatatagaccaaacagcattatattggaagaaaatgccatctaggactttcatagctacagaaaggaagtcagcacctggcttcaaagcttcaaaggacaggctgtctctattgttaggagttaatgcagctggtgactttaagttgaagtcaatgtccatttaccattcaggaaatcctaagacccttaggaattatgctaagactactctgcctgtgctctataaatgctatcaaacagcaacaaagtctgaatgacagcctatttatttatagcatggtttactgaatattttaagcccactcttgagacctactgctgagaagaaaaaagatttctcaaaatgttactgttcatggacaatgcacctggtcacccaagggctctgatggagatgtgcaaggagattattgttgttttcatgcctgctaacacaatgtccattctgcagcccatggatcaaggagtaatttcaactttcaagtcttattatttaagaaatacattttgtaaagctatacctgccttacagtcctcctgcctatctgatggatctaggcaaagtaaattgaaaaccttctggaaagagttcactattgtcaatgccatgaaaaacattcgtgattcatggaaggatgtcaatacatcaacattaacaggagtttggaagaagttgattccaatcctcatgagtgactttgagggattcagtggaggaagtaactgcagatatggtggaaatagcaagagaattagaatcataagtggaacctgaagatgtgagtgaattgctgccaactcatgataaaacttaaatagatggggagttgcttcttatggatgtgcaaagaacgtgatttcttgagatggaaactcctcctggtgaagatgctgtgaacattgttgaaatgacaagaagggatttagaatattacataaacttagttgataaagcagtgacagggttggagaggattgactccaattttgaaagaagttctaccatgggtaaaatgctatcaaacagcatcgcagccttcagagaaatttttcataaaaaaaggagtcaattgatgtggcaaacttcgttgttgtcttcttttttaaaattgccacagccacaccaaccttcagcagccaccaccctgatcagtcagcagccatcaacattgaagcaagcccctccaccagcaacaagattacaactcactaaaggctcagatgattgttagcttttttagtaataaagtatgcttaaattatgtacatattttagatataattctattgcacatttaatagactacagtgtagtgtagatataacttttatatgcactgggaaaccaagcaatttacgtgacacaatttgctttattacaatattcactttatttccattatctgaaatgaaacccacattatctttgaggtgtgcctgtattttgttcaggagggaactgaggaagacactcttatccaggatgagctgaaattgtttctcaagttgttcttgacaggggaaagagtctttggaggtcatgtttgaaatgagggtttgggactctatgaatttcaattatacatgtcctctctgctctgcctccagataataaatatacaatcatgtcatctgcaaacagagacaatttgacttcctctcttcctatttgaatatcctttatttctttctcttgcctgattgccctgtccagaacttccaatactatgttgaataggagtggtgagagagggcatccttgtcttgtgctggttttcaaagagaatgcttccggcttttgcccattcagtatgatattggctgtgggtttgtcctaaatagctcttattattttgagatacgttccatcaatacctagtttatggagagtttttagtatgaagggctgttgagttttatcgaaggccttttctgcatctattgaggtaatcatgtggttttggtcattggttctgtttacgtgacggattacgtttattgatttgcatatgttgaaccagccttccatcccagggaggaagccgacttgatcatagtggataagctttttgaggtgctgctagattcagtttgctagtattttattgaggatttttgcatcgatgttcatcagggatattggtctaaaattgtctttttttgttgcgtctctgccaggctttggtatcaggattatgctggcctcataaaatgagttagggaggagtccctctttttctattgcttggaatagtttcagaatgaatggtaccagctcctctttgtacctctggtagaatttggctgtgaatccgtctggtcttgggctttttttggttggtagactattaattactgcctcaatttcaaaacttgttcttgttctattcaggggttcgatttcttcctagtttagtcttgggagggtgtatgtgtccaggaatttatccatttcttctagattttctagtttatttgcctagaggtgtttatagtatagtactctctgttggtagtttgtatttctgtgggattagtggtaatatcccctttatcattttttattgcatctatttgattcttctttcttttcttctttattagtctggctagcggtctatttttttgatcttttcaaaaaaccggctcctggattcattgatttttttgaagggatttttgtgtctctgtctccttcagttctgctctgatcttagttatttcttgtcttctgctagcttttgaatttgtttgctcttgcttctctagttcatttaattgtgatgttagggtgttgattttagatcttccctgctttctcttatgggcatttagtgctataaatttccctctaaacactgcctccagataataaagaactacttagaataagtgacttttcataaagtgtcagtgttcagtctcttcttttttacagtaatgaactggtatttcctttacacatctttggatttattctgatttcttatgaaagagaaaacagggagcccaagtattaactgcaaggagaaccagatttcattaaacggtgacctggatgaattcctaatatcatatgctttattctttgcagagaagggcttatggtttgattttttcaaaaaatgctggctacttatccctcctttgacatcagtttggtttgccttcatatgtttggagtataacatgctttatttggcctttgggcttctcaagtttaaaaacatgcacttcattatatctgtaatggatattttgatagagtgatgaatatgctcttccattttgctgttctctaagattactgtggaaccatgattattgatggagaagaagctccagttgcctacacgttggatgataccaaacctgaaggcaactatgctgccataatggggtaaggcacaattatggtgttgtggctgctattcagtgttgacaagataatcacatactattaacaaatgtgccccaaactttgttaagtgattttttttttacccagtggtattatttttcaaattcagcggtacaaaaattattactggttcttttctaaataatgtcttccaatgaataaatatctaggtaggaagcagaataccaataacattttaaaatttttatgttagttttctattagtatttagtgttgggggtagacatatttaggtgacccatcttttgttgaaagcatgataaaaagacctgacttggggtgttttactaagagacttcttgtggaggctgtgtgggcatccatgttacttaaatgagatgctgagatttctgagtcccagtagagaagagccaagaccagcccagtcttcagctttccagggacgaccagcacgtgggaagggaagaccaggatatcctggcccagagaggtggtgacctggagtatccaaaattaagatgggcctcaggacatgtatgagtttatctcagagagagccaacagtcagaacagagagatcaaagctaattgttagttgaaagcaatcatggggctagaaatggagatggaatctagaaggttgggtgctagggagacaccatggtggagacaaaaccaaagagcaaggactggatgaaattggaagagctcagacatagccttaagtgggcatctgaggcccaagggttattcttattgaccaccagctgggtgaggggaagtgggtcagccatagtgttatccaaggcaaaaattatggccagtcatctacttttagtcgcttgattccttgaagttagaaagtgctcttcagtgtcagaaatttgatatgtaaatcataaaactttgaacgtaagaaaagctagtgtatagtttgtttcttttggttgacttaactgtgtaaactgggcacatgtgtagctacgaaaatgaggctaggatgaaaccaaccattaatttctcccctttttcttgtttatattctttagatttatcctggcccacaaagccagaaaactggcacgtcttaccaaagaggaaaggtaacaaaagaaatgctgcttctttcgtttcttccttcctttcccccccactccatccctccctcccttttctctttctttccttcttttctacctacttgcctgcctttcatttttacttaactttttaacttacggactgcctaattatatgtgtattgccagtgctacgtgtttgctatgttaattataagggtcttgttgtaaaagacatagtgctgataacttaagaaccaaagtattcaaattaatatttattgagtttattgtacataagacaccatgctaggggctacggagaatatgaaaatggatataacccaggggctgaaaatttgcttgtgaaggagataaaccagggagaaaaattactgtgttgtggggaagtctgctgtacacatactacatgaatgatgcataacaattacagattataggtacagtgggactaattcctctggaggtggcaatttcttcttgcaattagtgttcaccagtgccaattatttattcccacaccactgctaataacctatttaccaggaaagagctcctgaattatattatgatgcatgctttccgattccatcagggttctcctcaatgaccaatgttacctctgcacatagccagggccgtagcggtctgcctcggcctcttccctaaaaatgtccccactagaatataagatcatgaaggtaggatgttttgtctgattggctcactgctgggtttccagtgtctggaacaaatcttttcccactttgccttttgatcctgtttatggcttattcattttatactataataaaattttatctttttatgtaatcaaatttatccattttaaaaccatggtttctgagtatctatcatacatagaaaagactttctcattccaagataattttttagaaatcacccattcttccactcgttttatggtctgacctattatatgtaaatctttgatccttctgaaacatattttggtgtaagaaaataacgtaagcatcctactttatttctttcacgagcagctatttgtcccagtgccattttattgaaaactgtcttttccctgtgggttcaaaatgtccacctttatgaattctaaatttccttatatatttggttctacttctgtacttatttctttgctctttctatccattcctctgcttgtggcaagttacatcatttgtataaaaacaaagaaaaagacagaaagagagagaaagaagagagggagggagaagaacttaggcattttcataaacatttgtttcagaaacattttgttcataaacaaaagggctcctggatttaaaataataaaataataccatgattcaggcaacatgtcactttactttcttaaagacttaccagcaatcctgtgtgattaatatttgtgacctcaaagatttaagacatctgaaatggaacaaaatgccttgttttaaaaaattaaaatgaaatgctggagtggaatcaatggctcatggaatcttttttatgaggggataaatgcctctttcccactttttttttccctcccttctttcctttattttctcttttgtctcttttcattcacaggttgaagaaactttgtgaactctatgccaaggttctgggttccctagaagctctggaggtaaggctgcttcccaaccctatactaagggtgagaggcctttctttgtccccaagtgactagcagggataggttaatgcaagttgggtcctgaagttcatgtttttcccaatatatttgcagaggcatctacacaggactggtcagtttacaagtggttccagagagtgtgggccctggctgtgctggtggcaggtcagggaacttgcaatatgctgtggtttaggtgatgctacattgtccctgaattcagagtttcttcctgggagagggcattgggtcactctgcttccagttctgttaggggggtaaaagaggggagcttctactacccataggaagatcctagatcctggtagccaggatggggatgaaaagggctttttcccctctctggtgatcttgtaagaaggacagagtctcactcaggtacataaacctatacctaccccatcccccactgtctcacagtaaaaaaataagattacctgtccccactcctgcatgccctcttttctgccttgttttacccttgaacatgagagatgtaaagaagacaggctgtctgtctgtatgccagttgagttttctagacacctttggaagtagcctgagaaaacggtgatcttcaaatgaatcaagtagaactctaaggtggttaaaggtgggataggggcagggtagggggcatttggtgacagtcagagggcccaaagtactcataacaagtacccataatcacctccctcatcaatatttaaaatgatgaattggtgttctcatgacattcatcagactgctaagtttttaatgttttgacatagactatgtcaccttttgaaagtgattattaaatccaattatctgtgaagcatttgaagacaatggagaccaatgtacaaatgagcagttaatgcgtgagaaaagtctaatgaggaggctgagaatgtttaacttgttaagcctcttaaatccaagtctctgtagtatataccacaatctagttgagcagctacatgacttagtcctattactctaacacttactttgctcagctttggagtgacttgcttcctcctggttaagttgttgtgtctttcaaatttgtcatttttgttcactattttaaagcaaaattctctccctccctcctcgccccaccattgcagatcttctgtacttgatacaggtgaaacacatgctcttgatgtttcttggaattctttctcagcaaataaactagaacaattagagaaacaatattaatgaggaatatgttttgctttttttttttgctttcatataccaattagcaagtttaaatataggcatagcctccaggctcaaggatattgagtaaagtatcaagacaaaaaatacagtatatactcactaaaaacagaacttaacatctgttaaaaattattagtttttctgtttaaaaatgccattcagcatgatttataatcctttgggtatatacccagtaatgggattgctgggtcaaatgatatttctagttctagatccctgaggaatcgccacactgacttccacagtggttgaactagtttacagtcccaccaacagtgtaaaagacatatgcacacgtatgtttattgcggcactattcacaatagcaaagacttgaaaccaacccaaatgtccaacaatgatagactggattaagaaaatgtggcacatatacaccatggaatactatgcagccataaaaatgatgagttcatgtcctttgtagggacatggatgaagctggaaaccgtcattctcagcaaactatcgcagggacaaaaaaccaaacactgcatgttctcactcataggtgggaattgaacaatgagaacacatggacacaggaaggggaacatcacacactgggacctgttgtggggtggggggaggggggagggatagcatttggagatatacctaatgttaaatgacgagttactgggtgcagcacaccaacatggcacatgtatacatatgtaactaacctgcacgttgtgcacatgtaccctaaaacttaaagtataataaaaaaaaatgccattcagtgctagaggtctggagaataaagagtgtggagttgatttaaaaaaaaaagccattcaagatatttcaccctggtagatattcaagctttgtgaagttacattctgaggcactcccaggctaaagcagtttgttaattgaagttcctgcaacaactcgtgagatggttgtttggggaacttcagttgaaggggaaagcatttgtcctcatattttgaaaaaggctgatcatttttcatttgagaaagtctcttttcctaagaagggtgtgcatgattaattcctgatgataaaaataagttggtcctgtccttgtttgctcttggcatagagaaggccacttgttttctttttgctttggtgtctattttgtggaaggaagaaattcctgggaacaagatacattgaaagataaagtccaacttttcttctgattggctggagacagccagagaagcttgcttaggaggtggatgtagccgtcaggtgctggggcgtgtagcgtggtgataccacagaagacctggagccacttaacccatcaggcagaacctcataatcatactttgtaaataggatgccttacaaatgactgtccaaagtcagctgtgtgattgcaattcttttaaacaaaatgtttttcaaaatctccctttaaaacaaacattgttttcttaaaacttgctacgttgattttatcttttcgaagtaatgcttaatgataaagcttctgtttggttactttaaaaaagcatttgagctttacaaaatctctgccaatttttcctgttcgtgtcaaaaacatatttttcagaccaatagttgtttacaaataccaccatcaacagaagtgcttgcctgccacaaaaacatgtttgttcagcctccctcaagaaagctcacctccaccaaaacatgaacctgataatcctttttcttcaacagacatatttttctgtctttttttcctatccagtcactccagtaaacataaatccttttaaaaacttttcttgaaaccatcaggcactaaaactttttaataggtaaaaccaaggtaaaaatggaattagattatcgcaatttatgaacagtacttaagatacaaagaaaccaaatgaaaaaaacattctaagatctgaatttcttagaagcttattaccaaggacatttacctgcccaaagacatatctttaaaaacatcaggataatgcaactctatttccgaaatacattggtttgacaatacaaagcctactaaactgttcgatttattctaggctaaatagctttctctgagtctccttcaagtttttgttgctctatcttgcagccagtgcattatgaagaaaagaactggtgtgaggagcagtactctgggggctgctacacaacttatttcccccctgggatcctgactcaatatggaaggtagagtaaaagcatgctaagctgttacagaaatcccctgcacctgaatccaaaacctaaataggttcaggtagctcttctcccttgtttcttataaatacaaaaaaaaaaaaaaaaaacaacccaatttcctttgtatcttatgaatgaaatcgtgtatcttatgaatgaaatcattataattatacatacatcatggtgctgcttttccctggaagagcaattccaatcaatataaccatagaaggtttcagcataagaatagcattttaccccattcttcatgatatgattattacgcattgcatgcctgtatcaaaacacatcatgtacccatagatatatacacctactctgtacccataaaaattaaaaatcaaaaaagagtagcattttaggtagtccaagggttcacccaatgtcagaagaagtgtccttatactgagttaggactcagtaaaacttcctcaaatgccactgtacaactgccaacacggggacaaaattataaaaacaaaatgagttctagactgggcatgaagagacttgggtcccagctctgattctaccaataacaaactttgtcatgccaaacaggtcacttctcctttctgaacctcactttcttagcaagtggatgggaaagcacaaaatgatgaaaagtgagcaataatcagtatgctcaagaaagtatgagttttttttattttttgatcctaatccttagatgctgggaagtatgagttattttttaacatccttattgagacgtaattcacataccatacaattcacctattcaaaacggtgcacagttcaatggcttttagcattcacagcattatacatccaagtgtgttgttgtttagttaatttatttgatgacaataaatgaactaataatatagcagtgatttttatgactattatactattactaaaccaagcaataatttaatgccaaaagcttaatctaaacaggatgagaaatgtagactagtgagtcaaagactgttgaaagtatgcagcaaacagagggggtaagtggaaatggctaatcaatctgtccatgaaaactggtcgaataaggagtaaaacctgcttatcagaagatacgtaataactttggttagcactttctttacctgcttaaagatggcaaaatattatccaagagaacattctggggccaaggggcagcacctgataagctgctgggtcattaagttaatttttagatatgctgactgtgttactctattttcacactgctgataaagacatacctgagaccgggcaatttacaaaagtaagaggtttattggacttacagttctacatggctggggaggcttcacaatcatggcaaaaggcaaggaggagcaagtcacatcttacgtcgatggcagcaggcaaagagagagcttgtgcaaagaaactcccgtttttaaaaccatcagatcttgtgagatccattcattatcaccagaacagcacaggaaagacccccgcccataattcactcatctcccactgggtccctcccacaacacatgagaattatgggagctacaatatgagatttgagtggggacacagagccaaatcgtatcactgagtgtagaatatgtcaatggtatttgtttcattctgcatttattggctaagtgccaaccatttgcgaagcactgtgctgagaacttcaataccaaggacagcctccctgctgagaaggagctgacagtgttgagggctagggtggggatggggagaggacatgatatcaaaaattgactctaaagtactgacatatgtccctggaagggaataaggataaaggagggcactactgtatcaccactcagaatgttaccactgaggtaaatgctctaatacaggggcatagagataccactggaacacacagaggcacaggctagctttacttagagaaatctgggaaggcttcataatgcacataccacctgagggttgtaggaggcagagaaaggctattggggatgcagtctatgcagatggaatggcatgaggaaaacgctaggatcccacaggtttctggaaagtctggggaagaactttgcatggatggtgtattaggccattcttgcattgcttaaaataaatacctgagtctggggaacttataaagaaaaaaggtttaattggctcatagttctgcaggctatacaagcatggtgctggcatctgctcagtttctggtgaagcctcagggagctcacaatcatggcagaaggcaaagtgagaacaggcaagtcacatggcgaaagcaggaacaagcaagtgtggtggggagaggtaccatacactcttaacgtgaccagatcttgctagaactcactatcatgaagaaggcaccaagccatgagggatccgtccccatgatccaaacacctcccaccaggccccacctcaagcattggaaattacaattctacatgagatttgggcagggacaaatatcaaaatattatatcagatgggctatgggtgatattaaggacagaatggagaatcagatcaaagggggaggaagaacagtttgccctatatgacacattcaggaatacaaaacttgatatttcaacagagaacagctatcactgcattacttttgtttttggctttgttttaaatcagaagtgtgatatgattagatttctgaccacagagtggtgggttttatgctcaatttcataaataccttttggtttggggaacaaagaggacactaacctgaactggcctgatcctgaccacgtgagagaagcaagataaatcccattgtatctggcattggtggtgatacagtaatgccttcttttatctttattccttcccagggatatatgtcaggcttcctataactaccttcaatttttagggtagaaactaaggcacagcatagcttaacataattcccagcttgaacagagactacctgcccagaagacttcccttgacccttcagggccatggtatttaagatattgcaataagttttatattcagagccctgaaagttcacagtacatgttctgaaggaaaagagaagacagaattaccagtacaacttggtaaagaactaaatatacatttcttaagaaatgtttcttctggatagggtgaaaaaaatgattgtcgtgattatgcagtaaaactcataagccacaagaaatatatgtggagttcccctttatgatgtcctatatcttttgtaaatatatactgtctgttcacgcacctgcaaaagaaggggcaggtatttttcttacctggttgttggactctttttttcccttaaaggaacataatttccaaatgacaagtggcgggaaactatctctttgtttaaaattaattcttggttttcacatattctgatttatagtatgattagttctctaagcctttgttctgtcttctaatatttcattcttagggtctagccaggcctcctagaggtctccagctggggttagttttctccattgaaaaaaaagtaaacatgtagtgaaaaacggcattgtttaatcaacacggggaaagtcaatccaccttctcttgtaggaagggttccttcctgagtacccttaggctctctatatatttcatgtgttgtcatcaatatactaatacaggtgttcctcaaaatatgatggggttatatcccaataaacccaccataaattgaaaatattataagtggaaaatgcgcttaatacacctaatgtactgaatatcatagtttagcttagctaccttaaacgtgctcagaacacttatattagccgacagttgggcataatcatctaacagaaagcgtattttataatagagggttgaatatttcatgtcaagttttaaatacggtattgaaagtgaaagacagaatggttgtatgggtacttgaagtatggtttctactgaatgtgtattgttttaacaccatcataaagttaacaattatacgttggagaccatctgtattctatataatatctctccttgtattttcttctcctttttgtgatgactacaatcagagcaggtgaaagaaaacccaccaatgcaagccagctcatttggttttctaataaaaggcccagtggtgtacagtgttgactaagatggaacatggatgttagttcttgacatcgcttatcagatataagagaaccatgagacaggatgaataatggcatgttgacggtgctttccttatggtatttttgtcagagcaacaatgaactgcccctcttacaggccaagtgctatgacatttcagtcccttgtatagcatgtgggcagtctactaactattaaatattatagggtgatgatacaccaggcaaagaatataagataaaaatagagactttgacatctgttagacatggttcaaatcctggctttgctattttctaggagtgtggctcttggcatatcactgaacatttctccaagcctcagtcttctcatatgtaaaaatgagataatgataatagtagctacatcacagagttctttaatagattgaagaaataatgcagtagagagaggaagtataactaagtggttaagactgtaggttccagagtcagattgcctgtgttcaaataccaactctgctacttactagctgtgaccgagagcaaattactttgtctttgttgctggttaggttccaggaagcagaccctgaaacaacgattagcagacaggatatatattaaggcatgcccttaggattggcagctgtggaagggagaaggaagcaggagtgggcatagggagaacttgggctgcagtgcagttccagtgaaggcctcagctgaccccagaggaagttccagaactagaatggcccttcagagtgggaggtctcaagttggagcttgggaatcaggtatttacagcccgtggtgatcagtcactggatgcaactgctattggaaggaggcatgacctagtaggtaacatagttttttttagcagaggcaatctccaaagagggctgacatcagtaggccctcttctggcagcactcccagcagctgggaataagtctttcattcttgaagggggcctgcgtggttcatcacaatgtccaccacagtctacctccatattcttatctgcaaaatggtgataataatagtaccgacctcaccagtacaggcaagtgttcaaggaataggagttatggagccatagtcagactctcagatttgttaaatgttactgattgaaagggtcttagaaatcagtggaccattccctttaagaggcaaggaagccagagcacagtgagagtaagtgatttgccaagttcactagtggaatagccagtggggaattgggggcatgtatcaccttgccacagagccagtgagccataaagggagccatgtgactgggcttacacagtccctcacttcatgttgatgaagcaaatacataatttacgtccattaatgtcagctccttcacctgcaactcttggtgcaggagtgaactttggcttttattctattttgtttgtgacaaggatcatgtaagagctggaggaaccacataaacattattccaaaattgccaatgtccttcttgattgtttagaatctgtggaagctgaccagcattggtctttatgggaaaacttttctctgactctctgagactgaccacttttgcctctttggttttgttccaagggttctacgccagccagtggacaggatttactttgcaggcaccgagactgccacacactggagcggctacatggagggggctgtagaggccggggagagagcagcccgagaggtagggtctggggtcatagattatggggaaggaggcaactcatggtcctgacatgtaggtcaaagatatctgagagcctggagaccaactctccagtaacccccatcttaagacccataaaatactattttaactattgtctcaggtgaagtgaacaccttagcccgaagtaataatgaaaatacctaacatgtcacccgaagtaaaaagagcccatggggcaaacgatcaacctgactatacttgaaaggtaacctaggtctgatattctagaaccaaacatgcttctattaggactcaaaattcaattcatttcacaggaaagattttctgacagttcctctgatgtcatccctatttgaggtgtgttcataactattaaaatttatggtaagcctaatgattggaacctcttataccacaggagaaagaccttttggcgcctcttaaaggttgtatggagtgttctggcctttaccttggtgtttttgatggatatctcaagagacagttacttagtcctttagggagcagattagaagaaagatggtgtcacttttgctatttgccagtgtgttctttcatttcagatcctgcatgccatggggaagattccagaggatgaaatctggcagtcagaaccagagtctgtggtaggctatgttttatttcatgaaattagatatcttttctctaaacccattattttcaagaagagcacacttgtatatattcacataccttttcctaagtgattcaactaagtgatttaaacatgaatgtttaaataagtatcatgggttagggtagaggtgagagatttagatgaactttgataaatttgtagctgtcacattcattacagattattaggaaaaaatattttttgatgaggagggagacatttctcggagacttctaaaaataataactcaataaatgcctgtcaaataaatatctagcctggtgattctccacatgaggtaggaaaagaaaggaaagtgtgttagcatctcctgtccagggacaaacaaatggaatgaaatggagaatatttagattaaaattttatttttaatatactcatcatttttgtaataaaatcctaggaagttttcctggctggaaggagggatgcatagaggttagagtgcaaacgcactttagaggacaaagtcacaaaggtcagaattattgctctatccttttaagtgtgaagtcaaagagaataggcctgccactccacagtcattctcttagtgcttctgccagggatgggattgtgggctgtagggaccattgattcatttactaacaagtatttatggcacacgtgttctgtatcagccattgtggcaaaggcacagcagcatttttgtggagctcaacatctggtggagaatgcagatgataaccaaaaagtacagaacagtgaagaagacatgctgagaaaaaatgcaaaaggagaatgtcatcctaggctggggtctcaggaaagaaagcctccctgaggaagtgaagggtccagtgaggaagacagggtaaacagtataagcagagggaacatcgtgtttactggtctagacgttggcaagaatgggtcatgttcagagagctggagaaagtacagactttctggaataaagtgcacaagccctgtactaatacccaatgttttctgaacctaggatgtccctgcacagcccatcaccaccacctttttggagagacatttgccctccgtgccaggcctgctcaggctgattggattgaccaccatcttttcagcaacggctcttggcttcctggcccacaaaagggggctacttgtgagagtctaaagagagagggtgtctgtaatcacactctcttcttactgtatttgggatatgagtttggggaaagagttgcagtaaagttccatgaagacaaatagtgtggagtgaggcggggagcatgaagataaatccaactctgactgtaaaatacatggtatctctttctccgttgtggcccctgcttagtgtcccttacctggcttagcgttctgtttcaccagtttccaagtttattgccctcaaaatctttagaatagttaaattggcttgtttaaggttcttgctgccccacaacacaccttgcccatgcacaaggaatgaattttttcctaccattatggctttgtgcttgttcttcctcttacctgtaatagcctcaccttccctagttctttgcattcgtccttagaatactgtattgttacagctgaaagacagtaaagaccatttagtcctcaccttctgttttagagttgagcaaactgaagcccacagaggtggaacttaattacctaagagccacaataagccactggtatctgggggactagaacacaaatccaacgcttttcccacctctttggatgttttccccaattatcctccttcactccctgtcatagttaccgatggtgtcccgttgtgtgggtttactctgtgctaagttgtcttacacttctcaaatgctactcagtatatagccttaagtcttactgttttgtgcggtgtgtctccagctgattttaacttttttgatggtagaaattttatctcttcttccttttgtatcctccattgtatcttcatacaaaggacagtacacacttgggtaattaaaaataaaagttgattgaccata